European Patent Specification EP 3 368 089 B1, published November 5, 2025. Title: NANOPARTICLE FORMULATIONS FOR DELIVERY OF NUCLEIC ACID COMPLEXES. Applicant: RaNA Therapeutics, Inc. Application Not Yet Assigned. The sequence listing filed with the application follows.

SEQUENCE LISTING (868 sequences)

SEQ ID NO: 1 - DNA, 15 bp, Artificial Sequence
  Synthetic Oligonucleotide
tgacccaagggagac

SEQ ID NO: 2 - DNA, 15 bp, Artificial Sequence
  Synthetic Oligonucleotide
tggccactggccgca

SEQ ID NO: 3 - DNA, 15 bp, Artificial Sequence
  Synthetic Oligonucleotide
cggcgacccctggtg

SEQ ID NO: 4 - DNA, 15 bp, Artificial Sequence
  Synthetic Oligonucleotide
cgccctccagcgctg

SEQ ID NO: 5 - DNA, 15 bp, Artificial Sequence
  Synthetic Oligonucleotide
cgctccgccctccag

SEQ ID NO: 6 - DNA, 17 bp, Artificial Sequence
  Synthetic Oligonucleotide
tgacccaagggagaccc

SEQ ID NO: 7 - DNA, 17 bp, Artificial Sequence
  Synthetic Oligonucleotide
tggccactggccgcacc

SEQ ID NO: 8 - DNA, 17 bp, Artificial Sequence
  Synthetic Oligonucleotide
cggcgacccctggtgcc

SEQ ID NO: 9 - DNA, 17 bp, Artificial Sequence
  Synthetic Oligonucleotide
cgccctccagcgctgcc

SEQ ID NO: 10 - DNA, 17 bp, Artificial Sequence
  Synthetic Oligonucleotide
cgctccgccctccagcc

SEQ ID NO: 11 - DNA, 24 bp, Artificial Sequence
  Synthetic Oligonucleotide
tgacccaagggagacggaaaccac

SEQ ID NO: 12 - DNA, 24 bp, Artificial Sequence
  Synthetic Oligonucleotide
tggccactggccgcaggaaaccac

SEQ ID NO: 13 - DNA, 24 bp, Artificial Sequence
  Synthetic Oligonucleotide
cggcgacccctggtgggaaacctc

SEQ ID NO: 14 - DNA, 24 bp, Artificial Sequence
  Synthetic Oligonucleotide
cgccctccagcgctgggaaacctc

SEQ ID NO: 15 - DNA, 24 bp, Artificial Sequence
  Synthetic Oligonucleotide
cgctccgccctccagccaaaggtc

SEQ ID NO: 16 - DNA, 15 bp, Artificial Sequence
  Synthetic Oligonucleotide
ggtttttaaggcttt

SEQ ID NO: 17 - DNA, 15 bp, Artificial Sequence
  Synthetic Oligonucleotide
ggggtcttggcctga

SEQ ID NO: 18 - DNA, 15 bp, Artificial Sequence
  Synthetic Oligonucleotide
cataatgaagctggg

SEQ ID NO: 19 - DNA, 15 bp, Artificial Sequence
  Synthetic Oligonucleotide
aggaggcaacacatt

SEQ ID NO: 20 - DNA, 15 bp, Artificial Sequence
  Synthetic Oligonucleotide
attattttgcttttt

SEQ ID NO: 21 - DNA, 15 bp, Artificial Sequence
  Synthetic Oligonucleotide
cattttccctcctgg

SEQ ID NO: 22 - DNA, 15 bp, Artificial Sequence
  Synthetic Oligonucleotide
gtaggctacccttta

SEQ ID NO: 23 - DNA, 15 bp, Artificial Sequence
  Synthetic Oligonucleotide
gaggcttgttgcttt

SEQ ID NO: 24 - DNA, 15 bp, Artificial Sequence
  Synthetic Oligonucleotide
catgtatgatgttat

SEQ ID NO: 25 - DNA, 20 bp, Artificial Sequence
  Synthetic Oligonucleotide
tttttggtttttaaggcttt

SEQ ID NO: 26 - DNA, 20 bp, Artificial Sequence
  Synthetic Oligonucleotide
tttttggggtcttggcctga

SEQ ID NO: 27 - DNA, 20 bp, Artificial Sequence
  Synthetic Oligonucleotide
tttttcataatgaagctggg

SEQ ID NO: 28 - DNA, 20 bp, Artificial Sequence
  Synthetic Oligonucleotide
tttttaggaggcaacacatt

SEQ ID NO: 29 - DNA, 20 bp, Artificial Sequence
  Synthetic Oligonucleotide
tttttattattttgcttttt

SEQ ID NO: 30 - DNA, 20 bp, Artificial Sequence
  Synthetic Oligonucleotide
tttttcattttccctcctgg

SEQ ID NO: 31 - DNA, 20 bp, Artificial Sequence
  Synthetic Oligonucleotide
tttttgtaggctacccttta

SEQ ID NO: 32 - DNA, 20 bp, Artificial Sequence
  Synthetic Oligonucleotide
tttttgaggcttgttgcttt

SEQ ID NO: 33 - DNA, 20 bp, Artificial Sequence
  Synthetic Oligonucleotide
tttttcatgtatgatgttat

SEQ ID NO: 34 - DNA, 20 bp, Artificial Sequence
  Synthetic Oligonucleotide
cggcgcccgagagtccacat

SEQ ID NO: 35 - DNA, 20 bp, Artificial Sequence
  Synthetic Oligonucleotide
ccaggaggccggctactgcg

SEQ ID NO: 36 - DNA, 20 bp, Artificial Sequence
  Synthetic Oligonucleotide
ctgggctgggctgggtgacg

SEQ ID NO: 37 - DNA, 20 bp, Artificial Sequence
  Synthetic Oligonucleotide
acccgggtgagggtctgggc

SEQ ID NO: 38 - DNA, 20 bp, Artificial Sequence
  Synthetic Oligonucleotide
ccaactctgccggccgcggg

SEQ ID NO: 39 - DNA, 20 bp, Artificial Sequence
  Synthetic Oligonucleotide
acggcggccgcagagtgggg

SEQ ID NO: 40 - DNA, 20 bp, Artificial Sequence
  Synthetic Oligonucleotide
tcgatgtcggtgcgcaggcc

SEQ ID NO: 41 - DNA, 20 bp, Artificial Sequence
  Synthetic Oligonucleotide
ggcggggcgtgcaggtcgca

SEQ ID NO: 42 - DNA, 20 bp, Artificial Sequence
  Synthetic Oligonucleotide
acgttggttcgaacttgcgc

SEQ ID NO: 43 - DNA, 20 bp, Artificial Sequence
  Synthetic Oligonucleotide
ttccaaatctggttgaggcc

SEQ ID NO: 44 - DNA, 20 bp, Artificial Sequence
  Synthetic Oligonucleotide
agacactctgctttttgaca

SEQ ID NO: 45 - DNA, 20 bp, Artificial Sequence
  Synthetic Oligonucleotide
tttcctcaaattcatcaaat

SEQ ID NO: 46 - DNA, 20 bp, Artificial Sequence
  Synthetic Oligonucleotide
gggtggcccaaagttccaga

SEQ ID NO: 47 - DNA, 20 bp, Artificial Sequence
  Synthetic Oligonucleotide
tggtctcatctagagagcct

SEQ ID NO: 48 - DNA, 20 bp, Artificial Sequence
  Synthetic Oligonucleotide
ctctgctagtctttcatagg

SEQ ID NO: 49 - DNA, 20 bp, Artificial Sequence
  Synthetic Oligonucleotide
gctaaagagtccagcgtttc

SEQ ID NO: 50 - DNA, 21 bp, Artificial Sequence
  Synthetic Oligonucleotide
gcaaggtcttcaaaaaactct

SEQ ID NO: 51 - DNA, 22 bp, Artificial Sequence
  Synthetic Oligonucleotide
ctcaaacgtgtatggcttgtct

SEQ ID NO: 52 - DNA, 21 bp, Artificial Sequence
  Synthetic Oligonucleotide
cccaaaggagacatcatagtc

SEQ ID NO: 53 - DNA, 24 bp, Artificial Sequence
  Synthetic Oligonucleotide
cagtttgacagttaagacaccact

SEQ ID NO: 54 - DNA, 21 bp, Artificial Sequence
  Synthetic Oligonucleotide
ataggttcctagatctccacc

SEQ ID NO: 55 - DNA, 20 bp, Artificial Sequence
  Synthetic Oligonucleotide
ggcgtctgcttgttgatcac

SEQ ID NO: 56 - DNA, 23 bp, Artificial Sequence
  Synthetic Oligonucleotide
aagatagccagatttgcttgttt

SEQ ID NO: 57 - DNA, 24 bp, Artificial Sequence
  Synthetic Oligonucleotide
ggtccactacatacctggatggag

SEQ ID NO: 58 - DNA, 21 bp, Artificial Sequence
  Synthetic Oligonucleotide
cccagtccagtcataacgctt

SEQ ID NO: 59 - DNA, 22 bp, Artificial Sequence
  Synthetic Oligonucleotide
cgtgggagtacacccagttttt

SEQ ID NO: 60 - DNA, 18 bp, Artificial Sequence
  Synthetic Oligonucleotide
catggagggacacgccgt

SEQ ID NO: 61 - DNA, 22 bp, Artificial Sequence
  Synthetic Oligonucleotide
gtgagctctgcggccagcagct

SEQ ID NO: 62 - DNA, 21 bp, Artificial Sequence
  Synthetic Oligonucleotide
agtttggtttttaaggcttta

SEQ ID NO: 63 - DNA, 21 bp, Artificial Sequence
  Synthetic Oligonucleotide
taggccaaggaagacaagtcc

SEQ ID NO: 64 - DNA, 19 bp, Artificial Sequence
  Synthetic Oligonucleotide
tcaagcatcttttccggaa

SEQ ID NO: 65 - DNA, 21 bp, Artificial Sequence
  Synthetic Oligonucleotide
tccttaaaacggggctgggca

SEQ ID NO: 66 - DNA, 21 bp, Artificial Sequence
  Synthetic Oligonucleotide
ttggcctgatagcttttaatg

SEQ ID NO: 67 - DNA, 27 bp, Artificial Sequence
  Synthetic Oligonucleotide
cctcagctgcataatgaagctggggtc

SEQ ID NO: 68 - DNA, 25 bp, Artificial Sequence
  Synthetic Oligonucleotide
aacaacaacaacaacaaaaaacaga

SEQ ID NO: 69 - DNA, 26 bp, Artificial Sequence
  Synthetic Oligonucleotide
cctcaaaagcaggaataaaaaaaata

SEQ ID NO: 70 - DNA, 23 bp, Artificial Sequence
  Synthetic Oligonucleotide
gctgtgacacatagcccaactgt

SEQ ID NO: 71 - DNA, 25 bp, Artificial Sequence
  Synthetic Oligonucleotide
ggaggcaacacattctttctacaga

SEQ ID NO: 72 - DNA, 15 bp, Artificial Sequence
  Synthetic Oligonucleotide
ctattaatattactg

SEQ ID NO: 73 - DNA, 16 bp, Artificial Sequence
  Synthetic Oligonucleotide
cattatgtgtatgtat

SEQ ID NO: 74 - DNA, 15 bp, Artificial Sequence
  Synthetic Oligonucleotide
tttatctatgttatt

SEQ ID NO: 75 - DNA, 15 bp, Artificial Sequence
  Synthetic Oligonucleotide
ctaatttgaagttct

SEQ ID NO: 76 - DNA, 15 bp, Artificial Sequence
  Synthetic Oligonucleotide
ttcgaacttgcgcgg

SEQ ID NO: 77 - DNA, 14 bp, Artificial Sequence
  Synthetic Oligonucleotide
tagagagcctgggt

SEQ ID NO: 78 - DNA, 15 bp, Artificial Sequence
  Synthetic Oligonucleotide
acaccactcccaaag

SEQ ID NO: 79 - DNA, 15 bp, Artificial Sequence
  Synthetic Oligonucleotide
aggtccactacatac

SEQ ID NO: 80 - DNA, 15 bp, Artificial Sequence
  Synthetic Oligonucleotide
cgttaacctggatgg

SEQ ID NO: 81 - DNA, 15 bp, Artificial Sequence
  Synthetic Oligonucleotide
aaagccttaaaaacc

SEQ ID NO: 82 - DNA, 15 bp, Artificial Sequence
  Synthetic Oligonucleotide
tcaggccaagacccc

SEQ ID NO: 83 - DNA, 15 bp, Artificial Sequence
  Synthetic Oligonucleotide
cccagcttcattatg

SEQ ID NO: 84 - DNA, 15 bp, Artificial Sequence
  Synthetic Oligonucleotide
aatgtgttgcctcct

SEQ ID NO: 85 - DNA, 15 bp, Artificial Sequence
  Synthetic Oligonucleotide
aaaaagcaaaataat

SEQ ID NO: 86 - DNA, 15 bp, Artificial Sequence
  Synthetic Oligonucleotide
ccaggagggaaaatg

SEQ ID NO: 87 - DNA, 15 bp, Artificial Sequence
  Synthetic Oligonucleotide
taaagggtagcctac

SEQ ID NO: 88 - DNA, 15 bp, Artificial Sequence
  Synthetic Oligonucleotide
aaagcaacaagcctc

SEQ ID NO: 89 - DNA, 15 bp, Artificial Sequence
  Synthetic Oligonucleotide
ataacatcatacatg

SEQ ID NO: 90 - DNA, 15 bp, Artificial Sequence
  Synthetic Oligonucleotide
gatactatcttcctc

SEQ ID NO: 91 - DNA, 15 bp, Artificial Sequence
  Synthetic Oligonucleotide
atgggggacggggca

SEQ ID NO: 92 - DNA, 15 bp, Artificial Sequence
  Synthetic Oligonucleotide
ggttgagactgggtg

SEQ ID NO: 93 - DNA, 15 bp, Artificial Sequence
  Synthetic Oligonucleotide
agactgaagaggtgc

SEQ ID NO: 94 - DNA, 15 bp, Artificial Sequence
  Synthetic Oligonucleotide
cgggacggctgtgtt

SEQ ID NO: 95 - DNA, 15 bp, Artificial Sequence
  Synthetic Oligonucleotide
tctgtgtgggcagca

SEQ ID NO: 96 - DNA, 15 bp, Artificial Sequence
  Synthetic Oligonucleotide
aaagccttaaaaacc

SEQ ID NO: 97 - DNA, 15 bp, Artificial Sequence
  Synthetic Oligonucleotide
tcaggccaagacccc

SEQ ID NO: 98 - DNA, 15 bp, Artificial Sequence
  Synthetic Oligonucleotide
cccagcttcattatg

SEQ ID NO: 99 - DNA, 15 bp, Artificial Sequence
  Synthetic Oligonucleotide
aatgtgttgcctcct

SEQ ID NO: 100 - DNA, 15 bp, Artificial Sequence
  Synthetic Oligonucleotide
aaaaagcaaaataat

SEQ ID NO: 101 - DNA, 15 bp, Artificial Sequence
  Synthetic Oligonucleotide
ccaggagggaaaatg

SEQ ID NO: 102 - DNA, 15 bp, Artificial Sequence
  Synthetic Oligonucleotide
taaagggtagcctac

SEQ ID NO: 103 - DNA, 15 bp, Artificial Sequence
  Synthetic Oligonucleotide
aaagcaacaagcctc

SEQ ID NO: 104 - DNA, 15 bp, Artificial Sequence
  Synthetic Oligonucleotide
ataacatcatacatg

SEQ ID NO: 105 - DNA, 15 bp, Artificial Sequence
  Synthetic Oligonucleotide
gatactatcttcctc

SEQ ID NO: 106 - DNA, 15 bp, Artificial Sequence
  Synthetic Oligonucleotide
atgggggacggggca

SEQ ID NO: 107 - DNA, 15 bp, Artificial Sequence
  Synthetic Oligonucleotide
ggttgagactgggtg

SEQ ID NO: 108 - DNA, 15 bp, Artificial Sequence
  Synthetic Oligonucleotide
agactgaagaggtgc

SEQ ID NO: 109 - DNA, 15 bp, Artificial Sequence
  Synthetic Oligonucleotide
cgggacggctgtgtt

SEQ ID NO: 110 - DNA, 15 bp, Artificial Sequence
  Synthetic Oligonucleotide
tctgtgtgggcagca

SEQ ID NO: 111 - DNA, 15 bp, Artificial Sequence
  Synthetic Oligonucleotide
gaagaagaagaagaa

SEQ ID NO: 112 - DNA, 15 bp, Artificial Sequence
  Synthetic Oligonucleotide
ttcttcttcttcttc

SEQ ID NO: 113 - DNA, 20 bp, Artificial Sequence
  Synthetic Oligonucleotide
cggcgcccgagagtccacat

SEQ ID NO: 114 - DNA, 20 bp, Artificial Sequence
  Synthetic Oligonucleotide
acggcggccgcagagtgggg

SEQ ID NO: 115 - DNA, 26 bp, Artificial Sequence
  Synthetic Oligonucleotide
cctcaaaagcaggaataaaaaaaata

SEQ ID NO: 116 - DNA, 15 bp, Artificial Sequence
  Synthetic Oligonucleotide
atgggggacggggca

SEQ ID NO: 117 - DNA, 15 bp, Artificial Sequence
  Synthetic Oligonucleotide
ggttgagactgggtg

SEQ ID NO: 118 - DNA, 15 bp, Artificial Sequence
  Synthetic Oligonucleotide
atgggggacggggca

SEQ ID NO: 119 - DNA, 35 bp, Artificial Sequence
  Synthetic Oligonucleotide
tgacccaagggagactttttggtttttaaggcttt

SEQ ID NO: 120 - DNA, 35 bp, Artificial Sequence
  Synthetic Oligonucleotide
tggccactggccgcatttttggtttttaaggcttt

SEQ ID NO: 121 - DNA, 35 bp, Artificial Sequence
  Synthetic Oligonucleotide
cggcgacccctggtgtttttggtttttaaggcttt

SEQ ID NO: 122 - DNA, 35 bp, Artificial Sequence
  Synthetic Oligonucleotide
cgccctccagcgctgtttttggtttttaaggcttt

SEQ ID NO: 123 - DNA, 35 bp, Artificial Sequence
  Synthetic Oligonucleotide
cgctccgccctccagtttttggtttttaaggcttt

SEQ ID NO: 124 - DNA, 35 bp, Artificial Sequence
  Synthetic Oligonucleotide
tgacccaagggagactttttggggtcttggcctga

SEQ ID NO: 125 - DNA, 35 bp, Artificial Sequence
  Synthetic Oligonucleotide
tggccactggccgcatttttggggtcttggcctga

SEQ ID NO: 126 - DNA, 35 bp, Artificial Sequence
  Synthetic Oligonucleotide
cggcgacccctggtgtttttggggtcttggcctga

SEQ ID NO: 127 - DNA, 35 bp, Artificial Sequence
  Synthetic Oligonucleotide
cgccctccagcgctgtttttggggtcttggcctga

SEQ ID NO: 128 - DNA, 35 bp, Artificial Sequence
  Synthetic Oligonucleotide
cgctccgccctccagtttttggggtcttggcctga

SEQ ID NO: 129 - DNA, 35 bp, Artificial Sequence
  Synthetic Oligonucleotide
tgacccaagggagactttttcataatgaagctggg

SEQ ID NO: 130 - DNA, 35 bp, Artificial Sequence
  Synthetic Oligonucleotide
tggccactggccgcatttttcataatgaagctggg

SEQ ID NO: 131 - DNA, 35 bp, Artificial Sequence
  Synthetic Oligonucleotide
cggcgacccctggtgtttttcataatgaagctggg

SEQ ID NO: 132 - DNA, 35 bp, Artificial Sequence
  Synthetic Oligonucleotide
cgccctccagcgctgtttttcataatgaagctggg

SEQ ID NO: 133 - DNA, 35 bp, Artificial Sequence
  Synthetic Oligonucleotide
cgctccgccctccagtttttcataatgaagctggg

SEQ ID NO: 134 - DNA, 35 bp, Artificial Sequence
  Synthetic Oligonucleotide
tgacccaagggagactttttaggaggcaacacatt

SEQ ID NO: 135 - DNA, 35 bp, Artificial Sequence
  Synthetic Oligonucleotide
tggccactggccgcatttttaggaggcaacacatt

SEQ ID NO: 136 - DNA, 35 bp, Artificial Sequence
  Synthetic Oligonucleotide
cggcgacccctggtgtttttaggaggcaacacatt

SEQ ID NO: 137 - DNA, 35 bp, Artificial Sequence
  Synthetic Oligonucleotide
cgccctccagcgctgtttttaggaggcaacacatt

SEQ ID NO: 138 - DNA, 35 bp, Artificial Sequence
  Synthetic Oligonucleotide
cgctccgccctccagtttttaggaggcaacacatt

SEQ ID NO: 139 - DNA, 35 bp, Artificial Sequence
  Synthetic Oligonucleotide
tgacccaagggagactttttattattttgcttttt

SEQ ID NO: 140 - DNA, 35 bp, Artificial Sequence
  Synthetic Oligonucleotide
tggccactggccgcatttttattattttgcttttt

SEQ ID NO: 141 - DNA, 35 bp, Artificial Sequence
  Synthetic Oligonucleotide
cggcgacccctggtgtttttattattttgcttttt

SEQ ID NO: 142 - DNA, 35 bp, Artificial Sequence
  Synthetic Oligonucleotide
cgccctccagcgctgtttttattattttgcttttt

SEQ ID NO: 143 - DNA, 35 bp, Artificial Sequence
  Synthetic Oligonucleotide
cgctccgccctccagtttttattattttgcttttt

SEQ ID NO: 144 - DNA, 35 bp, Artificial Sequence
  Synthetic Oligonucleotide
tgacccaagggagactttttcattttccctcctgg

SEQ ID NO: 145 - DNA, 35 bp, Artificial Sequence
  Synthetic Oligonucleotide
tggccactggccgcatttttcattttccctcctgg

SEQ ID NO: 146 - DNA, 35 bp, Artificial Sequence
  Synthetic Oligonucleotide
cggcgacccctggtgtttttcattttccctcctgg

SEQ ID NO: 147 - DNA, 35 bp, Artificial Sequence
  Synthetic Oligonucleotide
cgccctccagcgctgtttttcattttccctcctgg

SEQ ID NO: 148 - DNA, 35 bp, Artificial Sequence
  Synthetic Oligonucleotide
cgctccgccctccagtttttcattttccctcctgg

SEQ ID NO: 149 - DNA, 35 bp, Artificial Sequence
  Synthetic Oligonucleotide
tgacccaagggagactttttgtaggctacccttta

SEQ ID NO: 150 - DNA, 35 bp, Artificial Sequence
  Synthetic Oligonucleotide
tggccactggccgcatttttgtaggctacccttta

SEQ ID NO: 151 - DNA, 35 bp, Artificial Sequence
  Synthetic Oligonucleotide
cggcgacccctggtgtttttgtaggctacccttta

SEQ ID NO: 152 - DNA, 35 bp, Artificial Sequence
  Synthetic Oligonucleotide
cgccctccagcgctgtttttgtaggctacccttta

SEQ ID NO: 153 - DNA, 35 bp, Artificial Sequence
  Synthetic Oligonucleotide
cgctccgccctccagtttttgtaggctacccttta

SEQ ID NO: 154 - DNA, 35 bp, Artificial Sequence
  Synthetic Oligonucleotide
tgacccaagggagactttttgaggcttgttgcttt

SEQ ID NO: 155 - DNA, 35 bp, Artificial Sequence
  Synthetic Oligonucleotide
tggccactggccgcatttttgaggcttgttgcttt

SEQ ID NO: 156 - DNA, 35 bp, Artificial Sequence
  Synthetic Oligonucleotide
cggcgacccctggtgtttttgaggcttgttgcttt

SEQ ID NO: 157 - DNA, 35 bp, Artificial Sequence
  Synthetic Oligonucleotide
cgccctccagcgctgtttttgaggcttgttgcttt

SEQ ID NO: 158 - DNA, 35 bp, Artificial Sequence
  Synthetic Oligonucleotide
cgctccgccctccagtttttgaggcttgttgcttt

SEQ ID NO: 159 - DNA, 35 bp, Artificial Sequence
  Synthetic Oligonucleotide
tgacccaagggagactttttcatgtatgatgttat

SEQ ID NO: 160 - DNA, 35 bp, Artificial Sequence
  Synthetic Oligonucleotide
tggccactggccgcatttttcatgtatgatgttat

SEQ ID NO: 161 - DNA, 35 bp, Artificial Sequence
  Synthetic Oligonucleotide
cggcgacccctggtgtttttcatgtatgatgttat

SEQ ID NO: 162 - DNA, 35 bp, Artificial Sequence
  Synthetic Oligonucleotide
cgccctccagcgctgtttttcatgtatgatgttat

SEQ ID NO: 163 - DNA, 35 bp, Artificial Sequence
  Synthetic Oligonucleotide
cgctccgccctccagtttttcatgtatgatgttat

SEQ ID NO: 164 - DNA, 25 bp, Artificial Sequence
  Synthetic Oligonucleotide
cgccctccagtttttggtttttaag

SEQ ID NO: 165 - DNA, 25 bp, Artificial Sequence
  Synthetic Oligonucleotide
cgccctccagtttttggggtcttgg

SEQ ID NO: 166 - DNA, 25 bp, Artificial Sequence
  Synthetic Oligonucleotide
cgccctccagtttttcataatgaag

SEQ ID NO: 167 - DNA, 25 bp, Artificial Sequence
  Synthetic Oligonucleotide
cgccctccagtttttaggaggcaac

SEQ ID NO: 168 - DNA, 25 bp, Artificial Sequence
  Synthetic Oligonucleotide
cgccctccagtttttattattttgc

SEQ ID NO: 169 - DNA, 25 bp, Artificial Sequence
  Synthetic Oligonucleotide
cgccctccagtttttcattttccct

SEQ ID NO: 170 - DNA, 25 bp, Artificial Sequence
  Synthetic Oligonucleotide
cgccctccagtttttgtaggctacc

SEQ ID NO: 171 - DNA, 25 bp, Artificial Sequence
  Synthetic Oligonucleotide
cgccctccagtttttgaggcttgtt

SEQ ID NO: 172 - DNA, 25 bp, Artificial Sequence
  Synthetic Oligonucleotide
cgccctccagtttttcatgtatgat

SEQ ID NO: 173 - DNA, 27 bp, Artificial Sequence
  Synthetic Oligonucleotide
tgacccaagggagactttttttttttt

SEQ ID NO: 174 - DNA, 27 bp, Artificial Sequence
  Synthetic Oligonucleotide
tggccactggccgcatttttttttttt

SEQ ID NO: 175 - DNA, 27 bp, Artificial Sequence
  Synthetic Oligonucleotide
cggcgacccctggtgtttttttttttt

SEQ ID NO: 176 - DNA, 27 bp, Artificial Sequence
  Synthetic Oligonucleotide
cgccctccagcgctgtttttttttttt

SEQ ID NO: 177 - DNA, 27 bp, Artificial Sequence
  Synthetic Oligonucleotide
cgctccgccctccagtttttttttttt

SEQ ID NO: 178 - DNA, 15 bp, Artificial Sequence
  Synthetic Oligonucleotide
aaaataaacaacaac

SEQ ID NO: 179 - DNA, 16 bp, Artificial Sequence
  Synthetic Oligonucleotide
aggaataaaaaaaata

SEQ ID NO: 180 - DNA, 15 bp, Artificial Sequence
  Synthetic Oligonucleotide
tcaaaagcaggaata

SEQ ID NO: 181 - DNA, 15 bp, Artificial Sequence
  Synthetic Oligonucleotide
actgtcctcaaaagc

SEQ ID NO: 182 - DNA, 15 bp, Artificial Sequence
  Synthetic Oligonucleotide
agcccaactgtcctc

SEQ ID NO: 183 - DNA, 15 bp, Artificial Sequence
  Synthetic Oligonucleotide
tgacacatagcccaa

SEQ ID NO: 184 - DNA, 15 bp, Artificial Sequence
  Synthetic Oligonucleotide
gagctgtgacacata

SEQ ID NO: 185 - DNA, 15 bp, Artificial Sequence
  Synthetic Oligonucleotide
tctgggcctgggctg

SEQ ID NO: 186 - DNA, 15 bp, Artificial Sequence
  Synthetic Oligonucleotide
ggtgagggtctgggc

SEQ ID NO: 187 - DNA, 15 bp, Artificial Sequence
  Synthetic Oligonucleotide
gggacccgggtgagg

SEQ ID NO: 188 - DNA, 15 bp, Artificial Sequence
  Synthetic Oligonucleotide
ccggccgcgggaccc

SEQ ID NO: 189 - DNA, 15 bp, Artificial Sequence
  Synthetic Oligonucleotide
caactctgccggccg

SEQ ID NO: 190 - DNA, 15 bp, Artificial Sequence
  Synthetic Oligonucleotide
agtggggccaactct

SEQ ID NO: 191 - DNA, 15 bp, Artificial Sequence
  Synthetic Oligonucleotide
ggccgcagagtgggg

SEQ ID NO: 192 - DNA, 15 bp, Artificial Sequence
  Synthetic Oligonucleotide
gccacggcggccgca

SEQ ID NO: 193 - DNA, 15 bp, Artificial Sequence
  Synthetic Oligonucleotide
gtgcgcaggccacgg

SEQ ID NO: 194 - DNA, 15 bp, Artificial Sequence
  Synthetic Oligonucleotide
gggggacggggcagg

SEQ ID NO: 195 - DNA, 15 bp, Artificial Sequence
  Synthetic Oligonucleotide
gggacggggcaggtt

SEQ ID NO: 196 - DNA, 15 bp, Artificial Sequence
  Synthetic Oligonucleotide
gacggggcaggttga

SEQ ID NO: 197 - DNA, 15 bp, Artificial Sequence
  Synthetic Oligonucleotide
cggggcaggttgaga

SEQ ID NO: 198 - DNA, 15 bp, Artificial Sequence
  Synthetic Oligonucleotide
gggcaggttgagact

SEQ ID NO: 199 - DNA, 15 bp, Artificial Sequence
  Synthetic Oligonucleotide
gcaggttgagactgg

SEQ ID NO: 200 - DNA, 15 bp, Artificial Sequence
  Synthetic Oligonucleotide
aggttgagactgggt

SEQ ID NO: 201 - DNA, 15 bp, Artificial Sequence
  Synthetic Oligonucleotide
ggaaaaattccagga

SEQ ID NO: 202 - DNA, 15 bp, Artificial Sequence
  Synthetic Oligonucleotide
aattccaggagggaa

SEQ ID NO: 203 - DNA, 15 bp, Artificial Sequence
  Synthetic Oligonucleotide
gagggaaaatgaatt

SEQ ID NO: 204 - DNA, 17 bp, Artificial Sequence
  Synthetic Oligonucleotide
gaaaatgaattgtcttc

SEQ ID NO: 205 - DNA, 15 bp, Artificial Sequence
  Synthetic Oligonucleotide
gggggacggggcagg

SEQ ID NO: 206 - DNA, 15 bp, Artificial Sequence
  Synthetic Oligonucleotide
gggacggggcaggtt

SEQ ID NO: 207 - DNA, 15 bp, Artificial Sequence
  Synthetic Oligonucleotide
gacggggcaggttga

SEQ ID NO: 208 - DNA, 15 bp, Artificial Sequence
  Synthetic Oligonucleotide
cggggcaggttgaga

SEQ ID NO: 209 - DNA, 15 bp, Artificial Sequence
  Synthetic Oligonucleotide
gggcaggttgagact

SEQ ID NO: 210 - DNA, 15 bp, Artificial Sequence
  Synthetic Oligonucleotide
gcaggttgagactgg

SEQ ID NO: 211 - DNA, 15 bp, Artificial Sequence
  Synthetic Oligonucleotide
aggttgagactgggt

SEQ ID NO: 212 - DNA, 15 bp, Artificial Sequence
  Synthetic Oligonucleotide
ggaaaaattccagga

SEQ ID NO: 213 - DNA, 15 bp, Artificial Sequence
  Synthetic Oligonucleotide
aattccaggagggaa

SEQ ID NO: 214 - DNA, 15 bp, Artificial Sequence
  Synthetic Oligonucleotide
gagggaaaatgaatt

SEQ ID NO: 215 - DNA, 17 bp, Artificial Sequence
  Synthetic Oligonucleotide
gaaaatgaattgtcttc

SEQ ID NO: 216 - DNA, 15 bp, Artificial Sequence
  Synthetic Oligonucleotide
ggtggtttcagttct

SEQ ID NO: 217 - DNA, 20 bp, Artificial Sequence
  Synthetic Oligonucleotide
tttttggtggtttcagttct

SEQ ID NO: 218 - DNA, 15 bp, Artificial Sequence
  Synthetic Oligonucleotide
agcgtgctatctggg

SEQ ID NO: 219 - DNA, 15 bp, Artificial Sequence
  Synthetic Oligonucleotide
tggcccagggactct

SEQ ID NO: 220 - DNA, 14 bp, Artificial Sequence
  Synthetic Oligonucleotide
tctgcggctctggc

SEQ ID NO: 221 - DNA, 15 bp, Artificial Sequence
  Synthetic Oligonucleotide
cggtccggctctggg

SEQ ID NO: 222 - DNA, 15 bp, Artificial Sequence
  Synthetic Oligonucleotide
tcatcccgggaagct

SEQ ID NO: 223 - DNA, 15 bp, Artificial Sequence
  Synthetic Oligonucleotide
ccccaagtccccgct

SEQ ID NO: 224 - DNA, 15 bp, Artificial Sequence
  Synthetic Oligonucleotide
ccaaccatgcaagca

SEQ ID NO: 225 - DNA, 17 bp, Artificial Sequence
  Synthetic Oligonucleotide
tggcccagggactcttc

SEQ ID NO: 226 - DNA, 18 bp, Artificial Sequence
  Synthetic Oligonucleotide
cggtccggctctgggttc

SEQ ID NO: 227 - DNA, 17 bp, Artificial Sequence
  Synthetic Oligonucleotide
ccaaccatgcaagcacc

SEQ ID NO: 228 - DNA, 26 bp, Artificial Sequence
  Synthetic Oligonucleotide
tggcccagggactctcacaaagtgac

SEQ ID NO: 229 - DNA, 26 bp, Artificial Sequence
  Synthetic Oligonucleotide
cggtccggctctgggaagaaactttc

SEQ ID NO: 230 - DNA, 26 bp, Artificial Sequence
  Synthetic Oligonucleotide
ccaaccatgcaagcactcaaagagtc

SEQ ID NO: 231 - DNA, 34 bp, Artificial Sequence
  Synthetic Oligonucleotide
tggcccagggactctttttggtggtttcagttct

SEQ ID NO: 232 - DNA, 35 bp, Artificial Sequence
  Synthetic Oligonucleotide
cggtccggctctgggtttttggtggtttcagttct

SEQ ID NO: 233 - DNA, 35 bp, Artificial Sequence
  Synthetic Oligonucleotide
ccaaccatgcaagcatttttggtggtttcagttct

SEQ ID NO: 234 - DNA, 24 bp, Artificial Sequence
  Synthetic Oligonucleotide
cagggactctttttggtggtttca

SEQ ID NO: 235 - DNA, 25 bp, Artificial Sequence
  Synthetic Oligonucleotide
cggctctgggtttttggtggtttca

SEQ ID NO: 236 - DNA, 25 bp, Artificial Sequence
  Synthetic Oligonucleotide
catgcaagcatttttggtggtttca

SEQ ID NO: 237 - DNA, 29 bp, Artificial Sequence
  Synthetic Oligonucleotide
tggcccagggactcggtggtttcagttct

SEQ ID NO: 238 - DNA, 30 bp, Artificial Sequence
  Synthetic Oligonucleotide
cggtccggctctggtggtggtttcagttct

SEQ ID NO: 239 - DNA, 30 bp, Artificial Sequence
  Synthetic Oligonucleotide
ccaaccatgcaagcaggtggtttcagttct

SEQ ID NO: 240 - DNA, 20 bp, Artificial Sequence
  Synthetic Oligonucleotide
tttttagataaaatattata

SEQ ID NO: 241 - DNA, 19 bp, Artificial Sequence
  Synthetic Oligonucleotide
tttttattcagataaaata

SEQ ID NO: 242 - DNA, 20 bp, Artificial Sequence
  Synthetic Oligonucleotide
tttttggtttatttaaaact

SEQ ID NO: 243 - DNA, 20 bp, Artificial Sequence
  Synthetic Oligonucleotide
tttttaaatttatattacat

SEQ ID NO: 244 - DNA, 20 bp, Artificial Sequence
  Synthetic Oligonucleotide
tttttcttaaatttatatta

SEQ ID NO: 245 - DNA, 20 bp, Artificial Sequence
  Synthetic Oligonucleotide
tttttcacaaaatgttcatt

SEQ ID NO: 246 - DNA, 15 bp, Artificial Sequence
  Synthetic Oligonucleotide
cctccgccttctccc

SEQ ID NO: 247 - DNA, 15 bp, Artificial Sequence
  Synthetic Oligonucleotide
tctggtcgggaaact

SEQ ID NO: 248 - DNA, 15 bp, Artificial Sequence
  Synthetic Oligonucleotide
gctacagccttttcc

SEQ ID NO: 249 - DNA, 16 bp, Artificial Sequence
  Synthetic Oligonucleotide
cctccgccttctcccc

SEQ ID NO: 250 - DNA, 17 bp, Artificial Sequence
  Synthetic Oligonucleotide
tctggtcgggaaactcc

SEQ ID NO: 251 - DNA, 16 bp, Artificial Sequence
  Synthetic Oligonucleotide
gctacagccttttccc

SEQ ID NO: 252 - DNA, 24 bp, Artificial Sequence
  Synthetic Oligonucleotide
cctccgccttctccctctttgatc

SEQ ID NO: 253 - DNA, 26 bp, Artificial Sequence
  Synthetic Oligonucleotide
tctggtcgggaaactcaattattgtc

SEQ ID NO: 254 - DNA, 24 bp, Artificial Sequence
  Synthetic Oligonucleotide
gctacagccttttccactttgttc

SEQ ID NO: 255 - DNA, 35 bp, Artificial Sequence
  Synthetic Oligonucleotide
cctccgccttctccctttttagataaaatattata

SEQ ID NO: 256 - DNA, 34 bp, Artificial Sequence
  Synthetic Oligonucleotide
tctggtcgggaaactttttagataaaatattata

SEQ ID NO: 257 - DNA, 35 bp, Artificial Sequence
  Synthetic Oligonucleotide
gctacagccttttcctttttagataaaatattata

SEQ ID NO: 258 - DNA, 35 bp, Artificial Sequence
  Synthetic Oligonucleotide
cctccgccttctccctttttggtttatttaaaact

SEQ ID NO: 259 - DNA, 34 bp, Artificial Sequence
  Synthetic Oligonucleotide
tctggtcgggaaactttttggtttatttaaaact

SEQ ID NO: 260 - DNA, 35 bp, Artificial Sequence
  Synthetic Oligonucleotide
gctacagccttttcctttttggtttatttaaaact

SEQ ID NO: 261 - DNA, 35 bp, Artificial Sequence
  Synthetic Oligonucleotide
cctccgccttctccctttttaaatttatattacat

SEQ ID NO: 262 - DNA, 34 bp, Artificial Sequence
  Synthetic Oligonucleotide
tctggtcgggaaactttttaaatttatattacat

SEQ ID NO: 263 - DNA, 35 bp, Artificial Sequence
  Synthetic Oligonucleotide
gctacagccttttcctttttaaatttatattacat

SEQ ID NO: 264 - DNA, 25 bp, Artificial Sequence
  Synthetic Oligonucleotide
gccttctccctttttagataaaata

SEQ ID NO: 265 - DNA, 24 bp, Artificial Sequence
  Synthetic Oligonucleotide
tcgggaaactttttagataaaata

SEQ ID NO: 266 - DNA, 25 bp, Artificial Sequence
  Synthetic Oligonucleotide
agccttttcctttttagataaaata

SEQ ID NO: 267 - DNA, 25 bp, Artificial Sequence
  Synthetic Oligonucleotide
gccttctccctttttggtttattta

SEQ ID NO: 268 - DNA, 24 bp, Artificial Sequence
  Synthetic Oligonucleotide
tcgggaaactttttggtttattta

SEQ ID NO: 269 - DNA, 25 bp, Artificial Sequence
  Synthetic Oligonucleotide
agccttttcctttttggtttattta

SEQ ID NO: 270 - DNA, 25 bp, Artificial Sequence
  Synthetic Oligonucleotide
gccttctccctttttaaatttatat

SEQ ID NO: 271 - DNA, 24 bp, Artificial Sequence
  Synthetic Oligonucleotide
tcgggaaactttttaaatttatat

SEQ ID NO: 272 - DNA, 25 bp, Artificial Sequence
  Synthetic Oligonucleotide
agccttttcctttttaaatttatat

SEQ ID NO: 273 - DNA, 15 bp, Artificial Sequence
  Synthetic Oligonucleotide
aggtgtgcactttta

SEQ ID NO: 274 - DNA, 15 bp, Artificial Sequence
  Synthetic Oligonucleotide
tcatttttaaggtgt

SEQ ID NO: 275 - DNA, 20 bp, Artificial Sequence
  Synthetic Oligonucleotide
tttttaggtgtgcactttta

SEQ ID NO: 276 - DNA, 19 bp, Artificial Sequence
  Synthetic Oligonucleotide
tttttcatttttaaggtgt

SEQ ID NO: 277 - DNA, 15 bp, Artificial Sequence
  Synthetic Oligonucleotide
cgcggtctcggcggt

SEQ ID NO: 278 - DNA, 15 bp, Artificial Sequence
  Synthetic Oligonucleotide
atcatccatggtgag

SEQ ID NO: 279 - DNA, 34 bp, Artificial Sequence
  Synthetic Oligonucleotide
cgcggtctcggcggtttttaggtgtgcactttta

SEQ ID NO: 280 - DNA, 35 bp, Artificial Sequence
  Synthetic Oligonucleotide
atcatccatggtgagtttttaggtgtgcactttta

SEQ ID NO: 281 - DNA, 33 bp, Artificial Sequence
  Synthetic Oligonucleotide
cgcggtctcggcggtttttcatttttaaggtgt

SEQ ID NO: 282 - DNA, 34 bp, Artificial Sequence
  Synthetic Oligonucleotide
atcatccatggtgagtttttcatttttaaggtgt

SEQ ID NO: 283 - DNA, 24 bp, Artificial Sequence
  Synthetic Oligonucleotide
tctcggcggtttttaggtgtgcac

SEQ ID NO: 284 - DNA, 25 bp, Artificial Sequence
  Synthetic Oligonucleotide
ccatggtgagtttttaggtgtgcac

SEQ ID NO: 285 - DNA, 23 bp, Artificial Sequence
  Synthetic Oligonucleotide
tctcggcggtttttcatttttaa

SEQ ID NO: 286 - DNA, 24 bp, Artificial Sequence
  Synthetic Oligonucleotide
ccatggtgagtttttcatttttaa

SEQ ID NO: 287 - DNA, 30 bp, Artificial Sequence
  Synthetic Oligonucleotide
cgcggtctcggcggtaggtgtgcactttta

SEQ ID NO: 288 - DNA, 30 bp, Artificial Sequence
  Synthetic Oligonucleotide
atcatccatggtgagaggtgtgcactttta

SEQ ID NO: 289 - DNA, 30 bp, Artificial Sequence
  Synthetic Oligonucleotide
cgcggtctcggcggttcatttttaaggtgt

SEQ ID NO: 290 - DNA, 30 bp, Artificial Sequence
  Synthetic Oligonucleotide
atcatccatggtgagtcatttttaaggtgt

SEQ ID NO: 291 - DNA, 15 bp, Artificial Sequence
  Synthetic Oligonucleotide
tggagccgagcgctg

SEQ ID NO: 292 - DNA, 15 bp, Artificial Sequence
  Synthetic Oligonucleotide
gggcctgcccctttg

SEQ ID NO: 293 - DNA, 15 bp, Artificial Sequence
  Synthetic Oligonucleotide
ccccaagtcacctga

SEQ ID NO: 294 - DNA, 15 bp, Artificial Sequence
  Synthetic Oligonucleotide
gacatcaatacctaa

SEQ ID NO: 295 - DNA, 15 bp, Artificial Sequence
  Synthetic Oligonucleotide
aaactttaccaagtc

SEQ ID NO: 296 - DNA, 17 bp, Artificial Sequence
  Synthetic Oligonucleotide
tggagccgagcgctgcc

SEQ ID NO: 297 - DNA, 17 bp, Artificial Sequence
  Synthetic Oligonucleotide
gggcctgcccctttgcc

SEQ ID NO: 298 - DNA, 17 bp, Artificial Sequence
  Synthetic Oligonucleotide
ccccaagtcacctgacc

SEQ ID NO: 299 - DNA, 17 bp, Artificial Sequence
  Synthetic Oligonucleotide
gacatcaatacctaacc

SEQ ID NO: 300 - DNA, 17 bp, Artificial Sequence
  Synthetic Oligonucleotide
aaactttaccaagtccc

SEQ ID NO: 301 - DNA, 24 bp, Artificial Sequence
  Synthetic Oligonucleotide
tggagccgagcgctgggaaaccac

SEQ ID NO: 302 - DNA, 24 bp, Artificial Sequence
  Synthetic Oligonucleotide
gggcctgcccctttgggaaaccac

SEQ ID NO: 303 - DNA, 24 bp, Artificial Sequence
  Synthetic Oligonucleotide
ccccaagtcacctgaggaaaccac

SEQ ID NO: 304 - DNA, 24 bp, Artificial Sequence
  Synthetic Oligonucleotide
gacatcaatacctaaggaaaccac

SEQ ID NO: 305 - DNA, 24 bp, Artificial Sequence
  Synthetic Oligonucleotide
aaactttaccaagtcggaaaccac

SEQ ID NO: 306 - DNA, 15 bp, Artificial Sequence
  Synthetic Oligonucleotide
actgcaatatatttc

SEQ ID NO: 307 - DNA, 15 bp, Artificial Sequence
  Synthetic Oligonucleotide
gtgttaaaattactt

SEQ ID NO: 308 - DNA, 20 bp, Artificial Sequence
  Synthetic Oligonucleotide
tttttactgcaatatatttc

SEQ ID NO: 309 - DNA, 20 bp, Artificial Sequence
  Synthetic Oligonucleotide
tttttgtgttaaaattactt

SEQ ID NO: 310 - DNA, 25 bp, Artificial Sequence
  Synthetic Oligonucleotide
ccgagcgctgtttttactgcaatat

SEQ ID NO: 311 - DNA, 25 bp, Artificial Sequence
  Synthetic Oligonucleotide
tgcccctttgtttttactgcaatat

SEQ ID NO: 312 - DNA, 25 bp, Artificial Sequence
  Synthetic Oligonucleotide
agtcacctgatttttactgcaatat

SEQ ID NO: 313 - DNA, 25 bp, Artificial Sequence
  Synthetic Oligonucleotide
caatacctaatttttactgcaatat

SEQ ID NO: 314 - DNA, 25 bp, Artificial Sequence
  Synthetic Oligonucleotide
ttaccaagtctttttactgcaatat

SEQ ID NO: 315 - DNA, 25 bp, Artificial Sequence
  Synthetic Oligonucleotide
ccgagcgctgtttttgtgttaaaat

SEQ ID NO: 316 - DNA, 25 bp, Artificial Sequence
  Synthetic Oligonucleotide
tgcccctttgtttttgtgttaaaat

SEQ ID NO: 317 - DNA, 25 bp, Artificial Sequence
  Synthetic Oligonucleotide
agtcacctgatttttgtgttaaaat

SEQ ID NO: 318 - DNA, 25 bp, Artificial Sequence
  Synthetic Oligonucleotide
caatacctaatttttgtgttaaaat

SEQ ID NO: 319 - DNA, 25 bp, Artificial Sequence
  Synthetic Oligonucleotide
ttaccaagtctttttgtgttaaaat

SEQ ID NO: 320 - DNA, 15 bp, Artificial Sequence
  Synthetic Oligonucleotide
tgtctgtagctccag

SEQ ID NO: 321 - DNA, 15 bp, Artificial Sequence
  Synthetic Oligonucleotide
tagctccagtgaggc

SEQ ID NO: 322 - DNA, 15 bp, Artificial Sequence
  Synthetic Oligonucleotide
tttcttctcccacca

SEQ ID NO: 323 - DNA, 17 bp, Artificial Sequence
  Synthetic Oligonucleotide
tgtctgtagctccagcc

SEQ ID NO: 324 - DNA, 17 bp, Artificial Sequence
  Synthetic Oligonucleotide
tagctccagtgaggccc

SEQ ID NO: 325 - DNA, 17 bp, Artificial Sequence
  Synthetic Oligonucleotide
tttcttctcccaccacc

SEQ ID NO: 326 - DNA, 24 bp, Artificial Sequence
  Synthetic Oligonucleotide
tgtctgtagctccagggaaaccac

SEQ ID NO: 327 - DNA, 24 bp, Artificial Sequence
  Synthetic Oligonucleotide
tagctccagtgaggcggaaaccac

SEQ ID NO: 328 - DNA, 24 bp, Artificial Sequence
  Synthetic Oligonucleotide
tttcttctcccaccaggaaaccac

SEQ ID NO: 329 - DNA, 20 bp, Artificial Sequence
  Synthetic Oligonucleotide
tttttgtgtgatctcttagc

SEQ ID NO: 330 - DNA, 20 bp, Artificial Sequence
  Synthetic Oligonucleotide
tttttgtgatctcttagcag

SEQ ID NO: 331 - DNA, 20 bp, Artificial Sequence
  Synthetic Oligonucleotide
ttttttgatctcttagcaga

SEQ ID NO: 332 - DNA, 15 bp, Artificial Sequence
  Synthetic Oligonucleotide
atttctctcaatcct

SEQ ID NO: 333 - DNA, 15 bp, Artificial Sequence
  Synthetic Oligonucleotide
ggcgtgtatattttt

SEQ ID NO: 334 - DNA, 15 bp, Artificial Sequence
  Synthetic Oligonucleotide
ggttatcgccctccc

SEQ ID NO: 335 - DNA, 15 bp, Artificial Sequence
  Synthetic Oligonucleotide
acgacttccgccgcc

SEQ ID NO: 336 - DNA, 17 bp, Artificial Sequence
  Synthetic Oligonucleotide
atttctctcaatcctcc

SEQ ID NO: 337 - DNA, 17 bp, Artificial Sequence
  Synthetic Oligonucleotide
ggcgtgtatatttttcc

SEQ ID NO: 338 - DNA, 17 bp, Artificial Sequence
  Synthetic Oligonucleotide
ggttatcgccctccccc

SEQ ID NO: 339 - DNA, 17 bp, Artificial Sequence
  Synthetic Oligonucleotide
acgacttccgccgcccc

SEQ ID NO: 340 - DNA, 24 bp, Artificial Sequence
  Synthetic Oligonucleotide
atttctctcaatcctggaaaccac

SEQ ID NO: 341 - DNA, 24 bp, Artificial Sequence
  Synthetic Oligonucleotide
ggcgtgtatatttttggaaaccac

SEQ ID NO: 342 - DNA, 24 bp, Artificial Sequence
  Synthetic Oligonucleotide
ggttatcgccctcccggaaaccac

SEQ ID NO: 343 - DNA, 24 bp, Artificial Sequence
  Synthetic Oligonucleotide
acgacttccgccgccggaaaccac

SEQ ID NO: 344 - DNA, 20 bp, Artificial Sequence
  Synthetic Oligonucleotide
ttttttaatttttttttaaa

SEQ ID NO: 345 - DNA, 20 bp, Artificial Sequence
  Synthetic Oligonucleotide
tttttatatgcaaaaaagaa

SEQ ID NO: 346 - DNA, 20 bp, Artificial Sequence
  Synthetic Oligonucleotide
tttttcaaaatatgggccaa

SEQ ID NO: 347 - DNA, 15 bp, Artificial Sequence
  Synthetic Oligonucleotide
ttcaccacatgtaaa

SEQ ID NO: 348 - DNA, 19 bp, Artificial Sequence
  Synthetic Oligonucleotide
ttttttcaccacatgtaaa

SEQ ID NO: 349 - DNA, 17 bp, Artificial Sequence
  Synthetic Oligonucleotide
aaatcagggcagaatgt

SEQ ID NO: 350 - DNA, 19 bp, Artificial Sequence
  Synthetic Oligonucleotide
aaatcagggcagaatgtcc

SEQ ID NO: 351 - DNA, 26 bp, Artificial Sequence
  Synthetic Oligonucleotide
aaatcagggcagaatgtccaaaggtc

SEQ ID NO: 352 - DNA, 36 bp, Artificial Sequence
  Synthetic Oligonucleotide
aaatcagggcagaatgtttttttcaccacatgtaaa

SEQ ID NO: 353 - DNA, 15 bp, Artificial Sequence
  Synthetic Oligonucleotide
ttattgtctgagccc

SEQ ID NO: 354 - DNA, 18 bp, Artificial Sequence
  Synthetic Oligonucleotide
tttttattgtctgagccc

SEQ ID NO: 355 - DNA, 15 bp, Artificial Sequence
  Synthetic Oligonucleotide
tcaggtgacggatgt

SEQ ID NO: 356 - DNA, 17 bp, Artificial Sequence
  Synthetic Oligonucleotide
tcaggtgacggatgtcc

SEQ ID NO: 357 - DNA, 24 bp, Artificial Sequence
  Synthetic Oligonucleotide
tcaggtgacggatgtccaaaggtc

SEQ ID NO: 358 - DNA, 33 bp, Artificial Sequence
  Synthetic Oligonucleotide
tcaggtgacggatgttttttattgtctgagccc

SEQ ID NO: 359 - DNA, 15 bp, Artificial Sequence
  Synthetic Oligonucleotide
tgtggggagctcggc

SEQ ID NO: 360 - DNA, 15 bp, Artificial Sequence
  Synthetic Oligonucleotide
ggggagctcggctgc

SEQ ID NO: 361 - DNA, 19 bp, Artificial Sequence
  Synthetic Oligonucleotide
tttttgtggggagctcggc

SEQ ID NO: 362 - DNA, 19 bp, Artificial Sequence
  Synthetic Oligonucleotide
ttttggggagctcggctgc

SEQ ID NO: 363 - DNA, 15 bp, Artificial Sequence
  Synthetic Oligonucleotide
ttgtccaagggcagg

SEQ ID NO: 364 - DNA, 15 bp, Artificial Sequence
  Synthetic Oligonucleotide
tcgatgagtgtgtgc

SEQ ID NO: 365 - DNA, 15 bp, Artificial Sequence
  Synthetic Oligonucleotide
agaagaaaaaccacg

SEQ ID NO: 366 - DNA, 15 bp, Artificial Sequence
  Synthetic Oligonucleotide
aatatgatttcttcc

SEQ ID NO: 367 - DNA, 15 bp, Artificial Sequence
  Synthetic Oligonucleotide
gagatgggggacatg

SEQ ID NO: 368 - DNA, 15 bp, Artificial Sequence
  Synthetic Oligonucleotide
ttcagtttattcaag

SEQ ID NO: 369 - DNA, 15 bp, Artificial Sequence
  Synthetic Oligonucleotide
ctgtctccacttttt

SEQ ID NO: 370 - DNA, 14 bp, Artificial Sequence
  Synthetic Oligonucleotide
tggaataaaacggg

SEQ ID NO: 371 - DNA, 15 bp, Artificial Sequence
  Synthetic Oligonucleotide
acaattgagaaaaca

SEQ ID NO: 372 - DNA, 15 bp, Artificial Sequence
  Synthetic Oligonucleotide
cagttttaagtggag

SEQ ID NO: 373 - DNA, 15 bp, Artificial Sequence
  Synthetic Oligonucleotide
tgacaagaatgagac

SEQ ID NO: 374 - DNA, 15 bp, Artificial Sequence
  Synthetic Oligonucleotide
ccgggcgaggggagg

SEQ ID NO: 375 - DNA, 15 bp, Artificial Sequence
  Synthetic Oligonucleotide
ccgccggcctgcccg

SEQ ID NO: 376 - DNA, 15 bp, Artificial Sequence
  Synthetic Oligonucleotide
cgagcgcgtatcctg

SEQ ID NO: 377 - DNA, 15 bp, Artificial Sequence
  Synthetic Oligonucleotide
ctgcttctcctcagc

SEQ ID NO: 378 - DNA, 17 bp, Artificial Sequence
  Synthetic Oligonucleotide
ttttcagtttattcaag

SEQ ID NO: 379 - DNA, 19 bp, Artificial Sequence
  Synthetic Oligonucleotide
ttttctgtctccacttttt

SEQ ID NO: 380 - DNA, 18 bp, Artificial Sequence
  Synthetic Oligonucleotide
tttttggaataaaacggg

SEQ ID NO: 381 - DNA, 19 bp, Artificial Sequence
  Synthetic Oligonucleotide
ttttacaattgagaaaaca

SEQ ID NO: 382 - DNA, 19 bp, Artificial Sequence
  Synthetic Oligonucleotide
ttttcagttttaagtggag

SEQ ID NO: 383 - DNA, 19 bp, Artificial Sequence
  Synthetic Oligonucleotide
tttttgacaagaatgagac

SEQ ID NO: 384 - DNA, 15 bp, Artificial Sequence
  Synthetic Oligonucleotide
aacagtcataataat

SEQ ID NO: 385 - DNA, 15 bp, Artificial Sequence
  Synthetic Oligonucleotide
taatttaacagtcat

SEQ ID NO: 386 - DNA, 15 bp, Artificial Sequence
  Synthetic Oligonucleotide
gcacgctataaagca

SEQ ID NO: 387 - DNA, 15 bp, Artificial Sequence
  Synthetic Oligonucleotide
cccggggctgggctt

SEQ ID NO: 388 - DNA, 15 bp, Artificial Sequence
  Synthetic Oligonucleotide
ccccgctccgcctcc

SEQ ID NO: 389 - DNA, 15 bp, Artificial Sequence
  Synthetic Oligonucleotide
gcgcctccctgattt

SEQ ID NO: 390 - DNA, 15 bp, Artificial Sequence
  Synthetic Oligonucleotide
tcgccgcggtggctg

SEQ ID NO: 391 - DNA, 15 bp, Artificial Sequence
  Synthetic Oligonucleotide
cagcgaatggtcgcg

SEQ ID NO: 392 - DNA, 20 bp, Artificial Sequence
  Synthetic Oligonucleotide
tttttaacagtcataataat

SEQ ID NO: 393 - DNA, 19 bp, Artificial Sequence
  Synthetic Oligonucleotide
tttttaatttaacagtcat

SEQ ID NO: 394 - DNA, 15 bp, Artificial Sequence
  Synthetic Oligonucleotide
gcggcggctgctcta

SEQ ID NO: 395 - DNA, 15 bp, Artificial Sequence
  Synthetic Oligonucleotide
ttatcggccgctgcc

SEQ ID NO: 396 - DNA, 15 bp, Artificial Sequence
  Synthetic Oligonucleotide
gcgtcggggacggct

SEQ ID NO: 397 - DNA, 15 bp, Artificial Sequence
  Synthetic Oligonucleotide
gcggaggaaactgcg

SEQ ID NO: 398 - DNA, 15 bp, Artificial Sequence
  Synthetic Oligonucleotide
gccgcacgcccgaca

SEQ ID NO: 399 - DNA, 15 bp, Artificial Sequence
  Synthetic Oligonucleotide
cctgacccaccctcc

SEQ ID NO: 400 - DNA, 15 bp, Artificial Sequence
  Synthetic Oligonucleotide
agggcaggccgcggc

SEQ ID NO: 401 - DNA, 15 bp, Artificial Sequence
  Synthetic Oligonucleotide
ctgaatcaccccgcg

SEQ ID NO: 402 - DNA, 15 bp, Artificial Sequence
  Synthetic Oligonucleotide
ggccccgagctccgc

SEQ ID NO: 403 - DNA, 15 bp, Artificial Sequence
  Synthetic Oligonucleotide
gcggctgctctaata

SEQ ID NO: 404 - DNA, 15 bp, Artificial Sequence
  Synthetic Oligonucleotide
cgccgcggcatgtgg

SEQ ID NO: 405 - DNA, 15 bp, Artificial Sequence
  Synthetic Oligonucleotide
ccctcctcctcttgc

SEQ ID NO: 406 - DNA, 15 bp, Artificial Sequence
  Synthetic Oligonucleotide
ggccgcgggctcgtg

SEQ ID NO: 407 - DNA, 15 bp, Artificial Sequence
  Synthetic Oligonucleotide
gttatttttctctgt

SEQ ID NO: 408 - DNA, 15 bp, Artificial Sequence
  Synthetic Oligonucleotide
atttaaaatgtttta

SEQ ID NO: 409 - DNA, 15 bp, Artificial Sequence
  Synthetic Oligonucleotide
tctctgtccatttaa

SEQ ID NO: 410 - DNA, 15 bp, Artificial Sequence
  Synthetic Oligonucleotide
tcatttggtcatgtg

SEQ ID NO: 411 - DNA, 15 bp, Artificial Sequence
  Synthetic Oligonucleotide
tagttctctgtacat

SEQ ID NO: 412 - DNA, 15 bp, Artificial Sequence
  Synthetic Oligonucleotide
tctgctggctcaact

SEQ ID NO: 413 - DNA, 15 bp, Artificial Sequence
  Synthetic Oligonucleotide
atcatagaatagatt

SEQ ID NO: 414 - DNA, 15 bp, Artificial Sequence
  Synthetic Oligonucleotide
ttatcatagaataga

SEQ ID NO: 415 - DNA, 15 bp, Artificial Sequence
  Synthetic Oligonucleotide
aattgacatttagca

SEQ ID NO: 416 - DNA, 15 bp, Artificial Sequence
  Synthetic Oligonucleotide
gacatttagcatttt

SEQ ID NO: 417 - DNA, 15 bp, Artificial Sequence
  Synthetic Oligonucleotide
ttaaccattcaacac

SEQ ID NO: 418 - DNA, 15 bp, Artificial Sequence
  Synthetic Oligonucleotide
cttggccggggaact

SEQ ID NO: 419 - DNA, 15 bp, Artificial Sequence
  Synthetic Oligonucleotide
gccggggaactgccg

SEQ ID NO: 420 - DNA, 15 bp, Artificial Sequence
  Synthetic Oligonucleotide
cgcccggagccgcgc

SEQ ID NO: 421 - DNA, 17 bp, Artificial Sequence
  Synthetic Oligonucleotide
cttggccggggaactcc

SEQ ID NO: 422 - DNA, 16 bp, Artificial Sequence
  Synthetic Oligonucleotide
gccggggaactgccgc

SEQ ID NO: 423 - DNA, 16 bp, Artificial Sequence
  Synthetic Oligonucleotide
cgcccggagccgcgcc

SEQ ID NO: 424 - DNA, 24 bp, Artificial Sequence
  Synthetic Oligonucleotide
cttggccggggaactataaaattc

SEQ ID NO: 425 - DNA, 34 bp, Artificial Sequence
  Synthetic Oligonucleotide
cttggccggggaactttttgtcgttcagataaaa

SEQ ID NO: 426 - DNA, 32 bp, Artificial Sequence
  Synthetic Oligonucleotide
cttggccggggaactttttcagataaaatatt

SEQ ID NO: 427 - DNA, 30 bp, Artificial Sequence
  Synthetic Oligonucleotide
cttggccggggaactgtcgttcagataaaa

SEQ ID NO: 428 - DNA, 30 bp, Artificial Sequence
  Synthetic Oligonucleotide
cttggccggggaactttcagataaaatatt

SEQ ID NO: 429 - DNA, 24 bp, Artificial Sequence
  Synthetic Oligonucleotide
ccggggaactttttgtcgttcaga

SEQ ID NO: 430 - DNA, 21 bp, Artificial Sequence
  Synthetic Oligonucleotide
cggggaactttttcagataaa

SEQ ID NO: 431 - DNA, 19 bp, Artificial Sequence
  Synthetic Oligonucleotide
cggggaactgtcgttcaga

SEQ ID NO: 432 - DNA, 20 bp, Artificial Sequence
  Synthetic Oligonucleotide
ccggggaactttcagataaa

SEQ ID NO: 433 - DNA, 15 bp, Artificial Sequence
  Synthetic Oligonucleotide
gtcgttcagataaaa

SEQ ID NO: 434 - DNA, 15 bp, Artificial Sequence
  Synthetic Oligonucleotide
ttcagataaaatatt

SEQ ID NO: 435 - DNA, 20 bp, Artificial Sequence
  Synthetic Oligonucleotide
tttttgtcgttcagataaaa

SEQ ID NO: 436 - DNA, 18 bp, Artificial Sequence
  Synthetic Oligonucleotide
tttttcagataaaatatt

SEQ ID NO: 437 - DNA, 15 bp, Artificial Sequence
  Synthetic Oligonucleotide
ctccgcggccgctcc

SEQ ID NO: 438 - DNA, 15 bp, Artificial Sequence
  Synthetic Oligonucleotide
gcccacatgctactc

SEQ ID NO: 439 - DNA, 15 bp, Artificial Sequence
  Synthetic Oligonucleotide
tccgaacgcccacat

SEQ ID NO: 440 - DNA, 15 bp, Artificial Sequence
  Synthetic Oligonucleotide
cgaggactcggtggt

SEQ ID NO: 441 - DNA, 15 bp, Artificial Sequence
  Synthetic Oligonucleotide
ccagctccgcggccg

SEQ ID NO: 442 - DNA, 16 bp, Artificial Sequence
  Synthetic Oligonucleotide
ctccgcggccgctccc

SEQ ID NO: 443 - DNA, 16 bp, Artificial Sequence
  Synthetic Oligonucleotide
gcccacatgctactcc

SEQ ID NO: 444 - DNA, 24 bp, Artificial Sequence
  Synthetic Oligonucleotide
ctccgcggccgctcctcaaagatc

SEQ ID NO: 445 - DNA, 24 bp, Artificial Sequence
  Synthetic Oligonucleotide
gcccacatgctactcccaaaggtc

SEQ ID NO: 446 - DNA, 35 bp, Artificial Sequence
  Synthetic Oligonucleotide
ctccgcggccgctcctttttgggagggaacacact

SEQ ID NO: 447 - DNA, 35 bp, Artificial Sequence
  Synthetic Oligonucleotide
gcccacatgctactctttttgggagggaacacact

SEQ ID NO: 448 - DNA, 30 bp, Artificial Sequence
  Synthetic Oligonucleotide
ctccgcggccgctccgggagggaacacact

SEQ ID NO: 449 - DNA, 30 bp, Artificial Sequence
  Synthetic Oligonucleotide
gcccacatgctactcgggagggaacacact

SEQ ID NO: 450 - DNA, 20 bp, Artificial Sequence
  Synthetic Oligonucleotide
cggccgctccgggagggaac

SEQ ID NO: 451 - DNA, 20 bp, Artificial Sequence
  Synthetic Oligonucleotide
catgctactcgggagggaac

SEQ ID NO: 452 - DNA, 15 bp, Artificial Sequence
  Synthetic Oligonucleotide
gggagggaacacact

SEQ ID NO: 453 - DNA, 15 bp, Artificial Sequence
  Synthetic Oligonucleotide
ggggtcttcacctga

SEQ ID NO: 454 - DNA, 15 bp, Artificial Sequence
  Synthetic Oligonucleotide
ggctgttatatcatg

SEQ ID NO: 455 - DNA, 15 bp, Artificial Sequence
  Synthetic Oligonucleotide
ggcattttaagatgg

SEQ ID NO: 456 - DNA, 20 bp, Artificial Sequence
  Synthetic Oligonucleotide
tttttgggagggaacacact

SEQ ID NO: 457 - DNA, 20 bp, Artificial Sequence
  Synthetic Oligonucleotide
tttttggctgttatatcatg

SEQ ID NO: 458 - DNA, 18 bp, Artificial Sequence
  Synthetic Oligonucleotide
ttttttttttggttttcc

SEQ ID NO: 459 - DNA, 15 bp, Artificial Sequence
  Synthetic Oligonucleotide
tgtctcatttggaga

SEQ ID NO: 460 - DNA, 14 bp, Artificial Sequence
  Synthetic Oligonucleotide
ataatgaagctggg

SEQ ID NO: 461 - DNA, 15 bp, Artificial Sequence
  Synthetic Oligonucleotide
ttttccctcctggaa

SEQ ID NO: 462 - DNA, 15 bp, Artificial Sequence
  Synthetic Oligonucleotide
tgcataatgaagctg

SEQ ID NO: 463 - DNA, 15 bp, Artificial Sequence
  Synthetic Oligonucleotide
aaatccttcaaagaa

SEQ ID NO: 464 - DNA, 15 bp, Artificial Sequence
  Synthetic Oligonucleotide
ttggaagattttttg

SEQ ID NO: 465 - DNA, 15 bp, Artificial Sequence
  Synthetic Oligonucleotide
gcattcttgtagcag

SEQ ID NO: 466 - DNA, 15 bp, Artificial Sequence
  Synthetic Oligonucleotide
acaacaaaaaacaga

SEQ ID NO: 467 - DNA, 15 bp, Artificial Sequence
  Synthetic Oligonucleotide
tgaagctggggtctt

SEQ ID NO: 468 - DNA, 15 bp, Artificial Sequence
  Synthetic Oligonucleotide
cctgaaaacatttgt

SEQ ID NO: 469 - DNA, 15 bp, Artificial Sequence
  Synthetic Oligonucleotide
ttcattttccctcct

SEQ ID NO: 470 - DNA, 15 bp, Artificial Sequence
  Synthetic Oligonucleotide
ttattattattatat

SEQ ID NO: 471 - DNA, 15 bp, Artificial Sequence
  Synthetic Oligonucleotide
taactttgcatgaat

SEQ ID NO: 472 - DNA, 15 bp, Artificial Sequence
  Synthetic Oligonucleotide
atacaaacatgtatg

SEQ ID NO: 473 - DNA, 15 bp, Artificial Sequence
  Synthetic Oligonucleotide
attgtaaacctataa

SEQ ID NO: 474 - DNA, 15 bp, Artificial Sequence
  Synthetic Oligonucleotide
tggagttggggttat

SEQ ID NO: 475 - DNA, 15 bp, Artificial Sequence
  Synthetic Oligonucleotide
gttggggttatttag

SEQ ID NO: 476 - DNA, 13 bp, Artificial Sequence
  Synthetic Oligonucleotide
ctccgccctccag

SEQ ID NO: 477 - DNA, 11 bp, Artificial Sequence
  Synthetic Oligonucleotide
ccgccctccag

SEQ ID NO: 478 - DNA, 9 bp, Artificial Sequence
  Synthetic Oligonucleotide
gccctccag

SEQ ID NO: 479 - DNA, 15 bp, Artificial Sequence
  Synthetic Oligonucleotide
cccgctccgccctcc

SEQ ID NO: 480 - DNA, 13 bp, Artificial Sequence
  Synthetic Oligonucleotide
cgctccgccctcc

SEQ ID NO: 481 - DNA, 11 bp, Artificial Sequence
  Synthetic Oligonucleotide
ctccgccctcc

SEQ ID NO: 482 - DNA, 9 bp, Artificial Sequence
  Synthetic Oligonucleotide
ccgccctcc

SEQ ID NO: 483 - DNA, 13 bp, Artificial Sequence
  Synthetic Oligonucleotide
gccactggccgca

SEQ ID NO: 484 - DNA, 11 bp, Artificial Sequence
  Synthetic Oligonucleotide
cactggccgca

SEQ ID NO: 485 - DNA, 13 bp, Artificial Sequence
  Synthetic Oligonucleotide
gcgacccctggtg

SEQ ID NO: 486 - DNA, 11 bp, Artificial Sequence
  Synthetic Oligonucleotide
gacccctggtg

SEQ ID NO: 487 - DNA, 13 bp, Artificial Sequence
  Synthetic Oligonucleotide
ctggccgcaggca

SEQ ID NO: 488 - DNA, 13 bp, Artificial Sequence
  Synthetic Oligonucleotide
ggccactggccgc

SEQ ID NO: 489 - DNA, 13 bp, Artificial Sequence
  Synthetic Oligonucleotide
ctggtggccactg

SEQ ID NO: 490 - DNA, 13 bp, Artificial Sequence
  Synthetic Oligonucleotide
gacccctggtggc

SEQ ID NO: 491 - DNA, 13 bp, Artificial Sequence
  Synthetic Oligonucleotide
gcggcgacccctg

SEQ ID NO: 492 - DNA, 13 bp, Artificial Sequence
  Synthetic Oligonucleotide
gtgctgcggcgac

SEQ ID NO: 493 - DNA, 13 bp, Artificial Sequence
  Synthetic Oligonucleotide
gctgggtgctgcg

SEQ ID NO: 494 - DNA, 13 bp, Artificial Sequence
  Synthetic Oligonucleotide
ccagcgctgggtg

SEQ ID NO: 495 - DNA, 13 bp, Artificial Sequence
  Synthetic Oligonucleotide
gccctccagcgct

SEQ ID NO: 496 - DNA, 13 bp, Artificial Sequence
  Synthetic Oligonucleotide
cgcccgctccgcc

SEQ ID NO: 497 - DNA, 35 bp, Artificial Sequence; identical to SEQ ID NO: 142
  Synthetic Oligonucleotide

SEQ ID NO: 498 - DNA, 35 bp, Artificial Sequence; identical to SEQ ID NO: 143
  Synthetic Oligonucleotide

SEQ ID NO: 499 - DNA, 17 bp, Artificial Sequence
  Synthetic Oligonucleotide
caagtccagtttggttt

SEQ ID NO: 500 - DNA, 17 bp, Artificial Sequence
  Synthetic Oligonucleotide
gaataggccaaggaaga

SEQ ID NO: 501 - DNA, 17 bp, Artificial Sequence
  Synthetic Oligonucleotide
atcaagcatcttttccg

SEQ ID NO: 502 - DNA, 17 bp, Artificial Sequence
  Synthetic Oligonucleotide
ttaaaacggggctgggc

SEQ ID NO: 503 - DNA, 17 bp, Artificial Sequence
  Synthetic Oligonucleotide
gatagcttttaatgtcc

SEQ ID NO: 504 - DNA, 17 bp, Artificial Sequence
  Synthetic Oligonucleotide
agctggggtcttggcct

SEQ ID NO: 505 - DNA, 17 bp, Artificial Sequence
  Synthetic Oligonucleotide
cctcagctgcataatga

SEQ ID NO: 506 - DNA, 17 bp, Artificial Sequence
  Synthetic Oligonucleotide
caacaacaaaaaacaga

SEQ ID NO: 507 - DNA, 17 bp, Artificial Sequence
  Synthetic Oligonucleotide
aaaaaaataaacaacaa

SEQ ID NO: 508 - DNA, 17 bp, Artificial Sequence
  Synthetic Oligonucleotide
cctcaaaagcaggaata

SEQ ID NO: 509 - DNA, 17 bp, Artificial Sequence
  Synthetic Oligonucleotide
acacatagcccaactgt

SEQ ID NO: 510 - DNA, 17 bp, Artificial Sequence
  Synthetic Oligonucleotide
ctttctacagagctgtg

SEQ ID NO: 511 - DNA, 17 bp, Artificial Sequence
  Synthetic Oligonucleotide
gtaggaggcaacacatt

SEQ ID NO: 512 - DNA, 17 bp, Artificial Sequence
  Synthetic Oligonucleotide
cagaacttgggggcaag

SEQ ID NO: 513 - DNA, 17 bp, Artificial Sequence
  Synthetic Oligonucleotide
ccatagaaattaaaaat

SEQ ID NO: 514 - DNA, 17 bp, Artificial Sequence
  Synthetic Oligonucleotide
acaatccaaaaaatctt

SEQ ID NO: 515 - DNA, 17 bp, Artificial Sequence
  Synthetic Oligonucleotide
gtgagggaggaaatccg

SEQ ID NO: 516 - DNA, 17 bp, Artificial Sequence
  Synthetic Oligonucleotide
aagataaggggtatcat

SEQ ID NO: 517 - DNA, 17 bp, Artificial Sequence
  Synthetic Oligonucleotide
ggcataagacattataa

SEQ ID NO: 518 - DNA, 17 bp, Artificial Sequence
  Synthetic Oligonucleotide
tgttatattcaggtata

SEQ ID NO: 519 - DNA, 17 bp, Artificial Sequence
  Synthetic Oligonucleotide
tttgcttttttaaaggt

SEQ ID NO: 520 - DNA, 17 bp, Artificial Sequence
  Synthetic Oligonucleotide
tttttccttcttattat

SEQ ID NO: 521 - DNA, 17 bp, Artificial Sequence
  Synthetic Oligonucleotide
cattttccctcctggaa

SEQ ID NO: 522 - DNA, 17 bp, Artificial Sequence
  Synthetic Oligonucleotide
gaagagtgaagacaatt

SEQ ID NO: 523 - DNA, 17 bp, Artificial Sequence
  Synthetic Oligonucleotide
taaatccttcaaagaat

SEQ ID NO: 524 - DNA, 17 bp, Artificial Sequence
  Synthetic Oligonucleotide
tcatgtacttcttgcag

SEQ ID NO: 525 - DNA, 17 bp, Artificial Sequence
  Synthetic Oligonucleotide
ggttgaccagctgctct

SEQ ID NO: 526 - DNA, 17 bp, Artificial Sequence
  Synthetic Oligonucleotide
agatagaacagtgagca

SEQ ID NO: 527 - DNA, 17 bp, Artificial Sequence
  Synthetic Oligonucleotide
taatgtgtctcatttgg

SEQ ID NO: 528 - DNA, 17 bp, Artificial Sequence
  Synthetic Oligonucleotide
atttgtaggctaccctt

SEQ ID NO: 529 - DNA, 17 bp, Artificial Sequence
  Synthetic Oligonucleotide
gaaagaagcctgaaaac

SEQ ID NO: 530 - DNA, 17 bp, Artificial Sequence
  Synthetic Oligonucleotide
agaagtgcttacacttt

SEQ ID NO: 531 - DNA, 17 bp, Artificial Sequence
  Synthetic Oligonucleotide
tcaatgctaaagagctc

SEQ ID NO: 532 - DNA, 13 bp, Artificial Sequence
  Synthetic Oligonucleotide
agtctgggtgtcc

SEQ ID NO: 533 - DNA, 13 bp, Artificial Sequence
  Synthetic Oligonucleotide
ccgacagtctggg

SEQ ID NO: 534 - DNA, 13 bp, Artificial Sequence
  Synthetic Oligonucleotide
ctccgacagtctg

SEQ ID NO: 535 - DNA, 13 bp, Artificial Sequence
  Synthetic Oligonucleotide
gacagtctgggtg

SEQ ID NO: 536 - DNA, 11 bp, Artificial Sequence
  Synthetic Oligonucleotide
cagtctgggtg

SEQ ID NO: 537 - DNA, 15 bp, Artificial Sequence
  Synthetic Oligonucleotide
ctcagcctggccctg

SEQ ID NO: 538 - DNA, 15 bp, Artificial Sequence
  Synthetic Oligonucleotide
agttcaaggatcagc

SEQ ID NO: 539 - DNA, 15 bp, Artificial Sequence
  Synthetic Oligonucleotide
gctctccgacagtct

SEQ ID NO: 540 - DNA, 13 bp, Artificial Sequence
  Synthetic Oligonucleotide
tctccgacagtct

SEQ ID NO: 541 - DNA, 11 bp, Artificial Sequence
  Synthetic Oligonucleotide
tccgacagtct

SEQ ID NO: 542 - DNA, 15 bp, Artificial Sequence
  Synthetic Oligonucleotide
cggagctctccgaca

SEQ ID NO: 543 - DNA, 13 bp, Artificial Sequence
  Synthetic Oligonucleotide
gagctctccgaca

SEQ ID NO: 544 - DNA, 11 bp, Artificial Sequence
  Synthetic Oligonucleotide
gctctccgaca

SEQ ID NO: 545 - DNA, 15 bp, Artificial Sequence
  Synthetic Oligonucleotide
ctattccattttgga

SEQ ID NO: 546 - DNA, 13 bp, Artificial Sequence
  Synthetic Oligonucleotide
ctattccattttg

SEQ ID NO: 547 - DNA, 15 bp, Artificial Sequence
  Synthetic Oligonucleotide
attccattttggaaa

SEQ ID NO: 548 - DNA, 15 bp, Artificial Sequence
  Synthetic Oligonucleotide
ccattttggaaaggt

SEQ ID NO: 549 - DNA, 13 bp, Artificial Sequence
  Synthetic Oligonucleotide
ccattttggaaag

SEQ ID NO: 550 - DNA, 15 bp, Artificial Sequence
  Synthetic Oligonucleotide
cattttggaaaggtt

SEQ ID NO: 551 - DNA, 13 bp, Artificial Sequence
  Synthetic Oligonucleotide
cattttggaaagg

SEQ ID NO: 552 - DNA, 15 bp, Artificial Sequence
  Synthetic Oligonucleotide
ggaaaggtttattgt

SEQ ID NO: 553 - DNA, 22 bp, Artificial Sequence
  Synthetic Oligonucleotide
tccgacagtctccattttggaa

SEQ ID NO: 554 - DNA, 22 bp, Artificial Sequence
  Synthetic Oligonucleotide
gctctccgacaccattttggaa

SEQ ID NO: 555 - DNA, 22 bp, Artificial Sequence
  Synthetic Oligonucleotide
tccgacagtctcattttggaaa

SEQ ID NO: 556 - DNA, 22 bp, Artificial Sequence
  Synthetic Oligonucleotide
gctctccgacacattttggaaa

SEQ ID NO: 557 - DNA, 15 bp, Artificial Sequence
  Synthetic Oligonucleotide
cctcaaaagcaggaa

SEQ ID NO: 558 - DNA, 13 bp, Artificial Sequence
  Synthetic Oligonucleotide
cctcaaaagcagg

SEQ ID NO: 559 - DNA, 11 bp, Artificial Sequence
  Synthetic Oligonucleotide
cctcaaaagca

SEQ ID NO: 560 - DNA, 13 bp, Artificial Sequence
  Synthetic Oligonucleotide
tcaaaagcaggaa

SEQ ID NO: 561 - DNA, 11 bp, Artificial Sequence
  Synthetic Oligonucleotide
caaaagcagga

SEQ ID NO: 562 - DNA, 27 bp, Artificial Sequence
  Synthetic Oligonucleotide
ccgccctccagcctcaaaagcaggaat

SEQ ID NO: 563 - DNA, 25 bp, Artificial Sequence
  Synthetic Oligonucleotide
ccgccctccagcctcaaaagcagga

SEQ ID NO: 564 - DNA, 23 bp, Artificial Sequence
  Synthetic Oligonucleotide
ccgccctccagcctcaaaagcag

SEQ ID NO: 565 - DNA, 21 bp, Artificial Sequence
  Synthetic Oligonucleotide
ccgccctccagcctcaaaagc

SEQ ID NO: 566 - DNA, 25 bp, Artificial Sequence
  Synthetic Oligonucleotide
gccctccagcctcaaaagcaggaat

SEQ ID NO: 567 - DNA, 23 bp, Artificial Sequence
  Synthetic Oligonucleotide
gccctccagcctcaaaagcagga

SEQ ID NO: 568 - DNA, 21 bp, Artificial Sequence
  Synthetic Oligonucleotide
gccctccagcctcaaaagcag

SEQ ID NO: 569 - DNA, 19 bp, Artificial Sequence
  Synthetic Oligonucleotide
gccctccagcctcaaaagc

SEQ ID NO: 570 - DNA, 17 bp, Artificial Sequence
  Synthetic Oligonucleotide
ccctccagcctcaaaag

SEQ ID NO: 571 - DNA, 15 bp, Artificial Sequence
  Synthetic Oligonucleotide
cctccagcctcaaaa

SEQ ID NO: 572 - DNA, 21 bp, Artificial Sequence
  Synthetic Oligonucleotide
gccctccagtcaaaagcagga

SEQ ID NO: 573 - DNA, 19 bp, Artificial Sequence
  Synthetic Oligonucleotide
gccctccagcaaaagcagg

SEQ ID NO: 574 - DNA, 23 bp, Artificial Sequence
  Synthetic Oligonucleotide
ccgccctccagtcaaaagcagga

SEQ ID NO: 575 - DNA, 21 bp, Artificial Sequence
  Synthetic Oligonucleotide
ccgccctccagcaaaagcagg

SEQ ID NO: 576 - DNA, 13 bp, Artificial Sequence
  Synthetic Oligonucleotide
ctccgccctccag

SEQ ID NO: 577 - DNA, 11 bp, Artificial Sequence
  Synthetic Oligonucleotide
ccgccctccag

SEQ ID NO: 578 - DNA, 9 bp, Artificial Sequence
  Synthetic Oligonucleotide
gccctccag

SEQ ID NO: 579 - DNA, 15 bp, Artificial Sequence
  Synthetic Oligonucleotide
cccgctccgccctcc

SEQ ID NO: 580 - DNA, 13 bp, Artificial Sequence
  Synthetic Oligonucleotide
cgctccgccctcc

SEQ ID NO: 581 - DNA, 11 bp, Artificial Sequence
  Synthetic Oligonucleotide
ctccgccctcc

SEQ ID NO: 582 - DNA, 9 bp, Artificial Sequence
  Synthetic Oligonucleotide
ccgccctcc

SEQ ID NO: 583 - DNA, 15 bp, Artificial Sequence
  Synthetic Oligonucleotide
gcctttgagaaagca

SEQ ID NO: 584 - DNA, 15 bp, Artificial Sequence
  Synthetic Oligonucleotide
gactgtggggccttt

SEQ ID NO: 585 - DNA, 15 bp, Artificial Sequence
  Synthetic Oligonucleotide
aggaagtggaggact

SEQ ID NO: 586 - DNA, 15 bp, Artificial Sequence
  Synthetic Oligonucleotide
tgcattttcactgaa

SEQ ID NO: 587 - DNA, 15 bp, Artificial Sequence
  Synthetic Oligonucleotide
cattttcactgaagc

SEQ ID NO: 588 - DNA, 15 bp, Artificial Sequence
  Synthetic Oligonucleotide
actgaagcatttatt

SEQ ID NO: 589 - DNA, 15 bp, Artificial Sequence
  Synthetic Oligonucleotide
cacacaaatgtatgg

SEQ ID NO: 590 - DNA, 15 bp, Artificial Sequence
  Synthetic Oligonucleotide
ggattttattgacaa

SEQ ID NO: 591 - DNA, 15 bp, Artificial Sequence
  Synthetic Oligonucleotide
aaaacaacaaagttt

SEQ ID NO: 592 - DNA, 15 bp, Artificial Sequence
  Synthetic Oligonucleotide
agtgccataaaaagt

SEQ ID NO: 593 - DNA, 15 bp, Artificial Sequence
  Synthetic Oligonucleotide
tcaaatataaaaatt

SEQ ID NO: 594 - DNA, 15 bp, Artificial Sequence
  Synthetic Oligonucleotide
ttccccccacccacc

SEQ ID NO: 595 - DNA, 15 bp, Artificial Sequence
  Synthetic Oligonucleotide
catttgcttccaatt

SEQ ID NO: 596 - DNA, 15 bp, Artificial Sequence
  Synthetic Oligonucleotide
gctcaaccctttttc

SEQ ID NO: 597 - DNA, 15 bp, Artificial Sequence
  Synthetic Oligonucleotide
agacctactactctg

SEQ ID NO: 598 - DNA, 15 bp, Artificial Sequence
  Synthetic Oligonucleotide
ccctccaccggaagt

SEQ ID NO: 599 - DNA, 15 bp, Artificial Sequence
  Synthetic Oligonucleotide
gcccgcgctcgccgt

SEQ ID NO: 600 - DNA, 15 bp, Artificial Sequence
  Synthetic Oligonucleotide
acgccccctggcagc

SEQ ID NO: 601 - DNA, 15 bp, Artificial Sequence
  Synthetic Oligonucleotide
gctcagcccctcggc

SEQ ID NO: 602 - DNA, 15 bp, Artificial Sequence
  Synthetic Oligonucleotide
agcagaggaagatca

SEQ ID NO: 603 - DNA, 15 bp, Artificial Sequence
  Synthetic Oligonucleotide
cagaggaagatcaaa

SEQ ID NO: 604 - DNA, 15 bp, Artificial Sequence
  Synthetic Oligonucleotide
cagatttttgaaact

SEQ ID NO: 605 - DNA, 15 bp, Artificial Sequence
  Synthetic Oligonucleotide
cagactaattttttg

SEQ ID NO: 606 - DNA, 15 bp, Artificial Sequence
  Synthetic Oligonucleotide
tttttgctttttcat

SEQ ID NO: 607 - DNA, 15 bp, Artificial Sequence
  Synthetic Oligonucleotide
aattttttgcttttt

SEQ ID NO: 608 - DNA, 15 bp, Artificial Sequence
  Synthetic Oligonucleotide
atgtttggcaatact

SEQ ID NO: 609 - DNA, 15 bp, Artificial Sequence
  Synthetic Oligonucleotide
ttggcaatacttttt

SEQ ID NO: 610 - DNA, 15 bp, Artificial Sequence
  Synthetic Oligonucleotide
gctgccctggccccg

SEQ ID NO: 611 - DNA, 15 bp, Artificial Sequence
  Synthetic Oligonucleotide
cggacacacccctcg

SEQ ID NO: 612 - DNA, 15 bp, Artificial Sequence
  Synthetic Oligonucleotide
acgggacgcgagtcc

SEQ ID NO: 613 - DNA, 15 bp, Artificial Sequence
  Synthetic Oligonucleotide
gtctggggagaaagc

SEQ ID NO: 614 - DNA, 15 bp, Artificial Sequence
  Synthetic Oligonucleotide
ccactcggtgggtct

SEQ ID NO: 615 - DNA, 15 bp, Artificial Sequence
  Synthetic Oligonucleotide
tgatctgttatcatc

SEQ ID NO: 616 - DNA, 15 bp, Artificial Sequence
  Synthetic Oligonucleotide
ctgttatcatctgta

SEQ ID NO: 617 - DNA, 15 bp, Artificial Sequence
  Synthetic Oligonucleotide
gtgtataaagatttt

SEQ ID NO: 618 - DNA, 15 bp, Artificial Sequence
  Synthetic Oligonucleotide
caatttacattttag

SEQ ID NO: 619 - DNA, 15 bp, Artificial Sequence
  Synthetic Oligonucleotide
tacattttagaccat

SEQ ID NO: 620 - DNA, 15 bp, Artificial Sequence
  Synthetic Oligonucleotide
tgctataagatgtaa

SEQ ID NO: 621 - DNA, 15 bp, Artificial Sequence
  Synthetic Oligonucleotide
aaggaagccggcaag

SEQ ID NO: 622 - DNA, 15 bp, Artificial Sequence
  Synthetic Oligonucleotide
cgccacaactcattc

SEQ ID NO: 623 - DNA, 15 bp, Artificial Sequence
  Synthetic Oligonucleotide
atgggagcattgtgg

SEQ ID NO: 624 - DNA, 15 bp, Artificial Sequence
  Synthetic Oligonucleotide
cgcccgcccagcccc

SEQ ID NO: 625 - DNA, 15 bp, Artificial Sequence
  Synthetic Oligonucleotide
cccctcccccgcccg

SEQ ID NO: 626 - DNA, 15 bp, Artificial Sequence
  Synthetic Oligonucleotide
cttccgctgctgctg

SEQ ID NO: 627 - DNA, 15 bp, Artificial Sequence
  Synthetic Oligonucleotide
cttcttagtaccaac

SEQ ID NO: 628 - DNA, 15 bp, Artificial Sequence
  Synthetic Oligonucleotide
tttagagcaaaatcg

SEQ ID NO: 629 - DNA, 15 bp, Artificial Sequence
  Synthetic Oligonucleotide
ggtagttaaatgttt

SEQ ID NO: 630 - DNA, 15 bp, Artificial Sequence
  Synthetic Oligonucleotide
tacttaagaaagaga

SEQ ID NO: 631 - DNA, 15 bp, Artificial Sequence
  Synthetic Oligonucleotide
tatacttaagaaaga

SEQ ID NO: 632 - DNA, 15 bp, Artificial Sequence
  Synthetic Oligonucleotide
cgccgccgacgccgg

SEQ ID NO: 633 - DNA, 15 bp, Artificial Sequence
  Synthetic Oligonucleotide
ctctctccgagagga

SEQ ID NO: 634 - DNA, 15 bp, Artificial Sequence
  Synthetic Oligonucleotide
cgccccgccctcttg

SEQ ID NO: 635 - DNA, 15 bp, Artificial Sequence
  Synthetic Oligonucleotide
ccgcgcgctgctgca

SEQ ID NO: 636 - DNA, 15 bp, Artificial Sequence
  Synthetic Oligonucleotide
cactttcacagagag

SEQ ID NO: 637 - DNA, 16 bp, Artificial Sequence
  Synthetic Oligonucleotide
ctttcacatgtattaa

SEQ ID NO: 638 - DNA, 15 bp, Artificial Sequence
  Synthetic Oligonucleotide
atgtattaaaaaact

SEQ ID NO: 639 - DNA, 15 bp, Artificial Sequence
  Synthetic Oligonucleotide
gacatttttatgtaa

SEQ ID NO: 640 - DNA, 15 bp, Artificial Sequence
  Synthetic Oligonucleotide
catttttatgtaaat

SEQ ID NO: 641 - DNA, 15 bp, Artificial Sequence
  Synthetic Oligonucleotide
aaatttataaggcaa

SEQ ID NO: 642 - DNA, 15 bp, Artificial Sequence
  Synthetic Oligonucleotide
aggcaaactctttat

SEQ ID NO: 643 - DNA, 15 bp, Artificial Sequence
  Synthetic Oligonucleotide
gtctctggaacaatt

SEQ ID NO: 644 - DNA, 15 bp, Artificial Sequence
  Synthetic Oligonucleotide
cagttcaaacacaga

SEQ ID NO: 645 - DNA, 15 bp, Artificial Sequence
  Synthetic Oligonucleotide
caaacacagaagaga

SEQ ID NO: 646 - DNA, 15 bp, Artificial Sequence
  Synthetic Oligonucleotide
aacacagaagagatt

SEQ ID NO: 647 - DNA, 15 bp, Artificial Sequence
  Synthetic Oligonucleotide
gggggagaagaaagg

SEQ ID NO: 648 - DNA, 15 bp, Artificial Sequence
  Synthetic Oligonucleotide
tcgtttttttttctt

SEQ ID NO: 649 - DNA, 15 bp, Artificial Sequence
  Synthetic Oligonucleotide
cttttttttcttttt

SEQ ID NO: 650 - DNA, 15 bp, Artificial Sequence
  Synthetic Oligonucleotide
cctatgctatggtta

SEQ ID NO: 651 - DNA, 15 bp, Artificial Sequence
  Synthetic Oligonucleotide
agtttactgaaagaa

SEQ ID NO: 652 - DNA, 15 bp, Artificial Sequence
  Synthetic Oligonucleotide
actgaaagaaaaaaa

SEQ ID NO: 653 - DNA, 15 bp, Artificial Sequence
  Synthetic Oligonucleotide
ccttattcatatttt

SEQ ID NO: 654 - DNA, 15 bp, Artificial Sequence
  Synthetic Oligonucleotide
cttccttattcatat

SEQ ID NO: 655 - DNA, 15 bp, Artificial Sequence
  Synthetic Oligonucleotide
caatccttcaatatt

SEQ ID NO: 656 - DNA, 15 bp, Artificial Sequence
  Synthetic Oligonucleotide
ggcatttcattttac

SEQ ID NO: 657 - DNA, 15 bp, Artificial Sequence
  Synthetic Oligonucleotide
cattttacaaatatt

SEQ ID NO: 658 - DNA, 15 bp, Artificial Sequence
  Synthetic Oligonucleotide
gaaatgaaataagta

SEQ ID NO: 659 - DNA, 15 bp, Artificial Sequence
  Synthetic Oligonucleotide
agatatgcaagataa

SEQ ID NO: 660 - DNA, 15 bp, Artificial Sequence
  Synthetic Oligonucleotide
gcgggcccagcaggt

SEQ ID NO: 661 - DNA, 15 bp, Artificial Sequence
  Synthetic Oligonucleotide
cagtgagtgccgagt

SEQ ID NO: 662 - DNA, 15 bp, Artificial Sequence
  Synthetic Oligonucleotide
gcccgggcagtgagt

SEQ ID NO: 663 - DNA, 15 bp, Artificial Sequence
  Synthetic Oligonucleotide
tgtccgggcggcccg

SEQ ID NO: 664 - DNA, 15 bp, Artificial Sequence
  Synthetic Oligonucleotide
cgcgcgtgtgcgagt

SEQ ID NO: 665 - DNA, 15 bp, Artificial Sequence
  Synthetic Oligonucleotide
cttcagacaggctgc

SEQ ID NO: 666 - DNA, 15 bp, Artificial Sequence
  Synthetic Oligonucleotide
acctctgcacttcag

SEQ ID NO: 667 - DNA, 15 bp, Artificial Sequence
  Synthetic Oligonucleotide
cggcgcgggtccctt

SEQ ID NO: 668 - DNA, 15 bp, Artificial Sequence
  Synthetic Oligonucleotide
tggtattcgaattat

SEQ ID NO: 669 - DNA, 15 bp, Artificial Sequence
  Synthetic Oligonucleotide
cggcctgccctggta

SEQ ID NO: 670 - DNA, 15 bp, Artificial Sequence
  Synthetic Oligonucleotide
tcagagattatgaaa

SEQ ID NO: 671 - DNA, 15 bp, Artificial Sequence
  Synthetic Oligonucleotide
tgttttcagagatta

SEQ ID NO: 672 - DNA, 15 bp, Artificial Sequence
  Synthetic Oligonucleotide
catgtagaaatgctt

SEQ ID NO: 673 - DNA, 15 bp, Artificial Sequence
  Synthetic Oligonucleotide
aaacatgtagaaatg

SEQ ID NO: 674 - DNA, 15 bp, Artificial Sequence
  Synthetic Oligonucleotide
ttgataccatttatg

SEQ ID NO: 675 - DNA, 15 bp, Artificial Sequence
  Synthetic Oligonucleotide
gaactcaattattat

SEQ ID NO: 676 - DNA, 15 bp, Artificial Sequence
  Synthetic Oligonucleotide
aaaacgactccacaa

SEQ ID NO: 677 - DNA, 15 bp, Artificial Sequence
  Synthetic Oligonucleotide
ctccgaggaaaaacg

SEQ ID NO: 678 - DNA, 15 bp, Artificial Sequence
  Synthetic Oligonucleotide
gctccgaggaaaaac

SEQ ID NO: 679 - DNA, 15 bp, Artificial Sequence
  Synthetic Oligonucleotide
ctcggcgggagaaag

SEQ ID NO: 680 - DNA, 13 bp, Artificial Sequence
  Synthetic Oligonucleotide
gaaccgaaatttt

SEQ ID NO: 681 - DNA, 15 bp, Artificial Sequence
  Synthetic Oligonucleotide
gagaagggtgcagat

SEQ ID NO: 682 - DNA, 15 bp, Artificial Sequence
  Synthetic Oligonucleotide
ctctccagatgagaa

SEQ ID NO: 683 - DNA, 15 bp, Artificial Sequence
  Synthetic Oligonucleotide
caggggtccgctctc

SEQ ID NO: 684 - DNA, 15 bp, Artificial Sequence
  Synthetic Oligonucleotide
tccgggcagccaggg

SEQ ID NO: 685 - DNA, 15 bp, Artificial Sequence
  Synthetic Oligonucleotide
ggggctcgcctccgg

SEQ ID NO: 686 - DNA, 15 bp, Artificial Sequence
  Synthetic Oligonucleotide
cccccgggaaggggc

SEQ ID NO: 687 - DNA, 15 bp, Artificial Sequence
  Synthetic Oligonucleotide
cccaccccccgggaa

SEQ ID NO: 688 - DNA, 16 bp, Artificial Sequence
  Synthetic Oligonucleotide
gcgttgccgcccccac

SEQ ID NO: 689 - DNA, 15 bp, Artificial Sequence
  Synthetic Oligonucleotide
gctgggtcgcgcgtt

SEQ ID NO: 690 - DNA, 15 bp, Artificial Sequence
  Synthetic Oligonucleotide
gcgcaggaccgctgg

SEQ ID NO: 691 - DNA, 15 bp, Artificial Sequence
  Synthetic Oligonucleotide
aggagggagggtggg

SEQ ID NO: 692 - DNA, 15 bp, Artificial Sequence
  Synthetic Oligonucleotide
cgctggaggcggagg

SEQ ID NO: 693 - DNA, 15 bp, Artificial Sequence
  Synthetic Oligonucleotide
tggagccgagcgctg

SEQ ID NO: 694 - DNA, 15 bp, Artificial Sequence
  Synthetic Oligonucleotide
ctgcccctttgttgg

SEQ ID NO: 695 - DNA, 15 bp, Artificial Sequence
  Synthetic Oligonucleotide
ctccccgctgcgggc

SEQ ID NO: 696 - DNA, 15 bp, Artificial Sequence
  Synthetic Oligonucleotide
cggctcctcctcctc

SEQ ID NO: 697 - DNA, 15 bp, Artificial Sequence
  Synthetic Oligonucleotide
ggctcgctccttcgg

SEQ ID NO: 698 - DNA, 15 bp, Artificial Sequence
  Synthetic Oligonucleotide
tttgtgcgcgagaga

SEQ ID NO: 699 - DNA, 15 bp, Artificial Sequence
  Synthetic Oligonucleotide
acgactccacaactt

SEQ ID NO: 700 - DNA, 15 bp, Artificial Sequence
  Synthetic Oligonucleotide
gcccgcttccctgct

SEQ ID NO: 701 - DNA, 15 bp, Artificial Sequence
  Synthetic Oligonucleotide
cggccggctgctgct

SEQ ID NO: 702 - DNA, 15 bp, Artificial Sequence
  Synthetic Oligonucleotide
gcgggagaaagcccg

SEQ ID NO: 703 - DNA, 15 bp, Artificial Sequence
  Synthetic Oligonucleotide
cctcctcgcccctcg

SEQ ID NO: 704 - DNA, 15 bp, Artificial Sequence
  Synthetic Oligonucleotide
agaggctcctcctcg

SEQ ID NO: 705 - DNA, 15 bp, Artificial Sequence
  Synthetic Oligonucleotide
tcggcttctggagcc

SEQ ID NO: 706 - DNA, 15 bp, Artificial Sequence
  Synthetic Oligonucleotide
ccgtgattccccaat

SEQ ID NO: 707 - DNA, 15 bp, Artificial Sequence
  Synthetic Oligonucleotide
aggggggcgccgctc

SEQ ID NO: 708 - DNA, 15 bp, Artificial Sequence
  Synthetic Oligonucleotide
aaatgacccaaaaga

SEQ ID NO: 709 - DNA, 15 bp, Artificial Sequence
  Synthetic Oligonucleotide
gttttccgtttgcag

SEQ ID NO: 710 - DNA, 15 bp, Artificial Sequence
  Synthetic Oligonucleotide
ccaaacgctacagag

SEQ ID NO: 711 - DNA, 15 bp, Artificial Sequence
  Synthetic Oligonucleotide
caggcaccaactttg

SEQ ID NO: 712 - DNA, 15 bp, Artificial Sequence
  Synthetic Oligonucleotide
cctggaaggggcgcg

SEQ ID NO: 713 - DNA, 15 bp, Artificial Sequence
  Synthetic Oligonucleotide
cagtcaaagcgcaaa

SEQ ID NO: 714 - DNA, 15 bp, Artificial Sequence
  Synthetic Oligonucleotide
ccaaaaacaaaacag

SEQ ID NO: 715 - DNA, 15 bp, Artificial Sequence
  Synthetic Oligonucleotide
ttccgccaaaaacaa

SEQ ID NO: 716 - DNA, 15 bp, Artificial Sequence
  Synthetic Oligonucleotide
ggaggagggagggtg

SEQ ID NO: 717 - DNA, 15 bp, Artificial Sequence
  Synthetic Oligonucleotide
cgagcgctggaggcg

SEQ ID NO: 718 - DNA, 15 bp, Artificial Sequence
  Synthetic Oligonucleotide
cctgcccctttgttg

SEQ ID NO: 719 - DNA, 15 bp, Artificial Sequence
  Synthetic Oligonucleotide
ggcggctcctcctcc

SEQ ID NO: 720 - DNA, 15 bp, Artificial Sequence
  Synthetic Oligonucleotide
tagacacttccagaa

SEQ ID NO: 721 - DNA, 15 bp, Artificial Sequence
  Synthetic Oligonucleotide
ttccagaattgtcct

SEQ ID NO: 722 - DNA, 15 bp, Artificial Sequence
  Synthetic Oligonucleotide
cagaattgtccttta

SEQ ID NO: 723 - DNA, 15 bp, Artificial Sequence
  Synthetic Oligonucleotide
ctgctggaactcggc

SEQ ID NO: 724 - DNA, 15 bp, Artificial Sequence
  Synthetic Oligonucleotide
ggccaggctcagctg

SEQ ID NO: 725 - DNA, 15 bp, Artificial Sequence
  Synthetic Oligonucleotide
gcagccaggagcctg

SEQ ID NO: 726 - DNA, 15 bp, Artificial Sequence
  Synthetic Oligonucleotide
actcggccaggctca

SEQ ID NO: 727 - DNA, 15 bp, Artificial Sequence
  Synthetic Oligonucleotide
gctggcctgctggaa

SEQ ID NO: 728 - DNA, 15 bp, Artificial Sequence
  Synthetic Oligonucleotide
tttaaattgtatcgg

SEQ ID NO: 729 - DNA, 15 bp, Artificial Sequence
  Synthetic Oligonucleotide
attgtatcgggcaaa

SEQ ID NO: 730 - DNA, 15 bp, Artificial Sequence
  Synthetic Oligonucleotide
gattaaaacaaaaga

SEQ ID NO: 731 - DNA, 15 bp, Artificial Sequence
  Synthetic Oligonucleotide
aaaacaaaagaaacc

SEQ ID NO: 732 - DNA, 15 bp, Artificial Sequence
  Synthetic Oligonucleotide
gggataaaggaaggg

SEQ ID NO: 733 - DNA, 15 bp, Artificial Sequence
  Synthetic Oligonucleotide
cactgggataaagga

SEQ ID NO: 734 - DNA, 15 bp, Artificial Sequence
  Synthetic Oligonucleotide
gagccgcccgctttg

SEQ ID NO: 735 - DNA, 14 bp, Artificial Sequence
  Synthetic Oligonucleotide
tctgggccccactg

SEQ ID NO: 736 - DNA, 15 bp, Artificial Sequence
  Synthetic Oligonucleotide
caaaaggtcttagct

SEQ ID NO: 737 - DNA, 15 bp, Artificial Sequence
  Synthetic Oligonucleotide
tagctattattactg

SEQ ID NO: 738 - DNA, 15 bp, Artificial Sequence
  Synthetic Oligonucleotide
actgttgttgtttta

SEQ ID NO: 739 - DNA, 15 bp, Artificial Sequence
  Synthetic Oligonucleotide
accttagaggttgta

SEQ ID NO: 740 - DNA, 15 bp, Artificial Sequence
  Synthetic Oligonucleotide
tacctgaaattgcag

SEQ ID NO: 741 - DNA, 15 bp, Artificial Sequence
  Synthetic Oligonucleotide
gtcagaaaagctacc

SEQ ID NO: 742 - DNA, 15 bp, Artificial Sequence
  Synthetic Oligonucleotide
cacgcttggtgtgca

SEQ ID NO: 743 - DNA, 15 bp, Artificial Sequence
  Synthetic Oligonucleotide
ctgtgaatgtgtgaa

SEQ ID NO: 744 - DNA, 15 bp, Artificial Sequence
  Synthetic Oligonucleotide
aacaggaagcacctg

SEQ ID NO: 745 - DNA, 39 bp, Artificial Sequence
  Synthetic Oligonucleotide
cgctccgccctccagtttttttttaggaggcaacacatt

SEQ ID NO: 746 - DNA, 41 bp, Artificial Sequence
  Synthetic Oligonucleotide
cgctccgccctccagcctttttttttaggaggcaacacatt

SEQ ID NO: 747 - DNA, 15 bp, Homo sapiens
ctgttataagctttt

SEQ ID NO: 748 - DNA, 15 bp, Homo sapiens
gttataagctttttc

SEQ ID NO: 749 - DNA, 15 bp, Homo sapiens
tatctgttataagct

SEQ ID NO: 750 - DNA, 15 bp, Homo sapiens
agtagatgtttattt

SEQ ID NO: 751 - DNA, 15 bp, Homo sapiens
taggcaaaggaatag

SEQ ID NO: 752 - DNA, 15 bp, Homo sapiens
ggtaggcaaaggaat

SEQ ID NO: 753 - DNA, 15 bp, Homo sapiens
ggcaaaggaatagtt

SEQ ID NO: 754 - DNA, 15 bp, Homo sapiens
gaaatgacacccagt

SEQ ID NO: 755 - DNA, 15 bp, Homo sapiens
aaatgacacccagta

SEQ ID NO: 756 - DNA, 15 bp, Homo sapiens
ggcaatggaatgaaa

SEQ ID NO: 757 - DNA, 15 bp, Homo sapiens
caatggaatgaaatg

SEQ ID NO: 758 - DNA, 15 bp, Homo sapiens
atggaatgaaatgac

SEQ ID NO: 759 - DNA, 15 bp, Homo sapiens
gtttcaagtacccgc

SEQ ID NO: 760 - DNA, 15 bp, Homo sapiens
gaccggagaacgaaa

SEQ ID NO: 761 - DNA, 15 bp, Homo sapiens
ctttggaaggtgttt

SEQ ID NO: 762 - DNA, 15 bp, Homo sapiens
tttctttggaaggtg

SEQ ID NO: 763 - DNA, 15 bp, Homo sapiens
agttaatccccgccg

SEQ ID NO: 764 - DNA, 15 bp, Homo sapiens
tcctgcaaaatgtca

SEQ ID NO: 765 - DNA, 15 bp, Homo sapiens
ccccgcagtctccac

SEQ ID NO: 766 - DNA, 15 bp, Homo sapiens
tctccaccctcctcc

SEQ ID NO: 767 - DNA, 15 bp, Homo sapiens
gagcgccggcgactg

SEQ ID NO: 768 - DNA, 15 bp, Homo sapiens
aggatgtgcgccttc

SEQ ID NO: 769 - DNA, 14 bp, Homo sapiens
ggcgcagcgaggaa

SEQ ID NO: 770 - DNA, 15 bp, Homo sapiens
tttcactgacatctc

SEQ ID NO: 771 - DNA, 15 bp, Homo sapiens
ggtggtctgagcccc

SEQ ID NO: 772 - DNA, 15 bp, Homo sapiens
gggcctgccagggga

SEQ ID NO: 773 - DNA, 15 bp, Homo sapiens
accgagtgacagtcg

SEQ ID NO: 774 - DNA, 15 bp, Homo sapiens
gtctgggaccgagtg

SEQ ID NO: 775 - DNA, 15 bp, Homo sapiens
tgggaccgagtgaca

SEQ ID NO: 776 - DNA, 15 bp, Homo sapiens
gcagaggtgtgttca

SEQ ID NO: 777 - DNA, 15 bp, Homo sapiens
cggcagaggtgtgtt

SEQ ID NO: 778 - DNA, 15 bp, Homo sapiens
gggcagacggggtca

SEQ ID NO: 779 - DNA, 15 bp, Homo sapiens
ctctggtttggaaaa

SEQ ID NO: 780 - DNA, 15 bp, Homo sapiens
ctggtttggaaaaca

SEQ ID NO: 781 - DNA, 15 bp, Homo sapiens
gtttggaaaacaaaa

SEQ ID NO: 782 - DNA, 15 bp, Homo sapiens
ggaaaacaaaagaac

SEQ ID NO: 783 - DNA, 15 bp, Homo sapiens
gaaaacaaaagaacc

SEQ ID NO: 784 - DNA, 15 bp, Homo sapiens
tttggaaaacaaaag

SEQ ID NO: 785 - DNA, 15 bp, Homo sapiens
tggaaaacaaaagaa

SEQ ID NO: 786 - DNA, 15 bp, Homo sapiens
tctggggcagcagga

SEQ ID NO: 787 - DNA, 15 bp, Homo sapiens
atagaaaggaacctt

SEQ ID NO: 788 - DNA, 15 bp, Homo sapiens
tagaaaggaaccttg

SEQ ID NO: 789 - DNA, 15 bp, Homo sapiens
attaacaatccttcc

SEQ ID NO: 790 - DNA, 15 bp, Homo sapiens
cttccctgctaaatg

SEQ ID NO: 791 - DNA, 15 bp, Homo sapiens
ccctgctaaatgata

SEQ ID NO: 792 - DNA, 15 bp, Homo sapiens
tgatataaacataga

SEQ ID NO: 793 - DNA, 15 bp, Homo sapiens
tccccgggactgaac

SEQ ID NO: 794 - DNA, 16 bp, Homo sapiens
tacaacttctttgaat

SEQ ID NO: 795 - DNA, 15 bp, Homo sapiens
tctatcacttccccg

SEQ ID NO: 796 - DNA, 15 bp, Homo sapiens
tcctgggcacccgta

SEQ ID NO: 797 - DNA, 15 bp, Homo sapiens
tttctgtacacatca

SEQ ID NO: 798 - DNA, 15 bp, Homo sapiens
acagccactgaaaat

SEQ ID NO: 799 - DNA, 15 bp, Homo sapiens
ttcacagccactgaa

SEQ ID NO: 800 - DNA, 15 bp, Homo sapiens
taaagaaatgagttt

SEQ ID NO: 801 - DNA, 15 bp, Homo sapiens
acatttaaagaaatg

SEQ ID NO: 802 - DNA, 15 bp, Homo sapiens
aagaaatgagtttgt

SEQ ID NO: 803 - DNA, 15 bp, Homo sapiens
tgccattatgtttgc

SEQ ID NO: 804 - DNA, 15 bp, Homo sapiens
tcctgttgccattat

SEQ ID NO: 805 - DNA, 15 bp, Homo sapiens
gaaaatcctgttgcc

SEQ ID NO: 806 - DNA, 15 bp, Homo sapiens
ctgttgccattatgt

SEQ ID NO: 807 - DNA, 15 bp, Homo sapiens
tagaattgaagtaac

SEQ ID NO: 808 - DNA, 15 bp, Homo sapiens
tgaagtaacaatcaa

SEQ ID NO: 809 - DNA, 15 bp, Homo sapiens
aagtaacaatcaatt

SEQ ID NO: 810 - DNA, 15 bp, Homo sapiens
tcatcaagatttctt

SEQ ID NO: 811 - DNA, 15 bp, Homo sapiens
tatctagcccaatat

SEQ ID NO: 812 - DNA, 15 bp, Homo sapiens
ttctatctagcccaa

SEQ ID NO: 813 - DNA, 33 bp, Homo sapiens
ctccgccctccagtttttattattttgcttttt

SEQ ID NO: 814 - DNA, 31 bp, Homo sapiens
ccgccctccagtttttattattttgcttttt

SEQ ID NO: 815 - DNA, 29 bp, Homo sapiens
gccctccagtttttattattttgcttttt

SEQ ID NO: 816 - DNA, 33 bp, Homo sapiens
cgctccgccctccagtttttattattttgcttt

SEQ ID NO: 817 - DNA, 31 bp, Homo sapiens
cgctccgccctccagtttttattattttgct

SEQ ID NO: 818 - DNA, 29 bp, Homo sapiens
cgctccgccctccagtttttattattttg

SEQ ID NO: 819 - DNA, 31 bp, Homo sapiens
ctccgccctccagtttttattattttgcttt

SEQ ID NO: 820 - DNA, 27 bp, Homo sapiens
ccgccctccagtttttattattttgct

SEQ ID NO: 821 - DNA, 25 bp, Homo sapiens
gccctccagtttttattattttgct

SEQ ID NO: 822 - DNA, 23 bp, Homo sapiens
ccctccagtttttattattttgc

SEQ ID NO: 823 - DNA, 21 bp, Homo sapiens
cctccagtttttattattttg

SEQ ID NO: 824 - DNA, 29 bp, Homo sapiens
gctccgccctccagattattttgcttttt

SEQ ID NO: 825 - DNA, 27 bp, Homo sapiens
tccgccctccagattattttgcttttt

SEQ ID NO: 826 - DNA, 25 bp, Homo sapiens
cgccctccagattattttgcttttt

SEQ ID NO: 827 - DNA, 23 bp, Homo sapiens
ccctccagattattttgcttttt

SEQ ID NO: 828 - DNA, 27 bp, Homo sapiens
gctccgccctccagattattttgcttt

SEQ ID NO: 829 - DNA, 25 bp, Homo sapiens
gctccgccctccagattattttgct

SEQ ID NO: 830 - DNA, 23 bp, Homo sapiens
gctccgccctccagattattttg

SEQ ID NO: 831 - DNA, 25 bp, Homo sapiens
tccgccctccagattattttgcttt

SEQ ID NO: 832 - DNA, 21 bp, Homo sapiens
cgccctccagattattttgct

SEQ ID NO: 833 - DNA, 19 bp, Homo sapiens
gccctccagattattttgc

SEQ ID NO: 834 - DNA, 17 bp, Homo sapiens
ccctccagattattttg

SEQ ID NO: 835 - DNA, 15 bp, Homo sapiens
ctccagattattttg

SEQ ID NO: 836 - DNA, 35 bp, Homo sapiens; identical to SEQ ID NO: 143

SEQ ID NO: 837 - DNA, 28 bp, Mus musculus
agttcaaggatcagccattttggaaagg

SEQ ID NO: 838 - DNA, 25 bp, Mus musculus
tcaaggatcagccattttggaaagg

SEQ ID NO: 839 - DNA, 23 bp, Mus musculus
aaggatcagccattttggaaagg

SEQ ID NO: 840 - DNA, 21 bp, Mus musculus
ggatcagccattttggaaagg

SEQ ID NO: 841 - DNA, 25 bp, Mus musculus
agttcaaggatcagccattttggaa

SEQ ID NO: 842 - DNA, 23 bp, Mus musculus
agttcaaggatcagccattttgg

SEQ ID NO: 843 - DNA, 27 bp, Mus musculus
gttcaaggatcagccattttggaaagg

SEQ ID NO: 844 - DNA, 23 bp, Mus musculus
tcaaggatcagccattttggaaa

SEQ ID NO: 845 - DNA, 21 bp, Mus musculus
aaggatcagccattttggaaa

SEQ ID NO: 846 - DNA, 19 bp, Mus musculus
aggatcagccattttggaa

SEQ ID NO: 847 - DNA, 17 bp, Mus musculus
ggatcagccattttgga

SEQ ID NO: 848 - DNA, 28 bp, Mus musculus
ctccgacagtctgccattttggaaaggt

SEQ ID NO: 849 - DNA, 25 bp, Mus musculus
cgacagtctgccattttggaaaggt

SEQ ID NO: 850 - DNA, 23 bp, Mus musculus
acagtctgccattttggaaaggt

SEQ ID NO: 851 - DNA, 25 bp, Mus musculus
ctccgacagtctgccattttggaaa

SEQ ID NO: 852 - DNA, 23 bp, Mus musculus
ctccgacagtctgccattttgga

SEQ ID NO: 853 - DNA, 21 bp, Mus musculus
ctccgacagtctgccattttg

SEQ ID NO: 854 - DNA, 27 bp, Mus musculus
ctccgacagtctgccattttggaaagg

SEQ ID NO: 855 - DNA, 23 bp, Mus musculus
ccgacagtctgccattttggaaa

SEQ ID NO: 856 - DNA, 19 bp, Mus musculus
gacagtctgccattttgga

SEQ ID NO: 857 - DNA, 17 bp, Mus musculus
acagtctgccattttgg

SEQ ID NO: 858 - DNA, 30 bp, Mus musculus
cggagctctccgacacattttggaaaggtt

SEQ ID NO: 859 - DNA, 29 bp, Mus musculus
ggagctctccgacacattttggaaaggtt

SEQ ID NO: 860 - DNA, 25 bp, Mus musculus
agctctccgacacattttggaaagg

SEQ ID NO: 861 - DNA, 21 bp, Mus musculus
ctctccgacacattttggaaa

SEQ ID NO: 862 - DNA, 19 bp, Mus musculus
tctccgacacattttggaa

SEQ ID NO: 863 - DNA, 17 bp, Mus musculus
ctccgacacattttgga

SEQ ID NO: 864 - DNA, 15 bp, Mus musculus
tccgacacattttgg

SEQ ID NO: 865 - DNA, 15 bp, Homo sapiens
cgctccgccctccag

SEQ ID NO: 866 - DNA, 15 bp, Homo sapiens
attattttgcttttt

SEQ ID NO: 867 - RNA, 29 nt, Artificial Sequence
  Synthetic Oligonucleotide
aaaaaaaaaaaaaaaaaaaaaaaaaaaaa

SEQ ID NO: 868 - RNA, 11 nt, Artificial Sequence
  Synthetic Oligonucleotide
aaaaaaaaaaa